European Patent Application EP 4 711 385 A1, published March 18, 2026. Title: Dual antigen targeting protein complex comprising an antibody or an antigen-binding fragment thereof, and affibodies. Applicant: AbClon Inc. The sequence listing filed with the application follows.

SEQUENCE LISTING (148 sequences)

SEQ ID NO: 1 - protein, 58 aa, synthetic construct
VDNKFNKEVCRAMEEIGMLPNLNAHQLAAFIWSLPDDPSQSANLLAEAKKLNDAQAPK

SEQ ID NO: 2 - protein, 58 aa, synthetic construct
VDNKFNKEECSAMQEISMLPNLNPHQFAAFIWSLMDDPSQSANLLAEAKKLNDAQAPK

SEQ ID NO: 3 - protein, 5 aa, synthetic construct
NYGVH

SEQ ID NO: 4 - protein, 16 aa, synthetic construct
VIWSGGNTDYNTPFTS

SEQ ID NO: 5 - protein, 11 aa, synthetic construct
ALTYYDYEFAY

SEQ ID NO: 6 - protein, 11 aa, synthetic construct
RASQSIGTNIH

SEQ ID NO: 7 - protein, 7 aa, synthetic construct
YASESIS

SEQ ID NO: 8 - protein, 9 aa, synthetic construct
QQNNNWPTT

SEQ ID NO: 9 - protein, 446 aa, synthetic construct
QVQLKQSGPGLVQPSQSLSITCTVSGFSLTNYGVHWVRQSPGKGLEWLGVIWSGGNTDYNTPFTSRLSINKDNSKSQVFFKMNSLQSNDTAIYYCARALTYYDYEFAYWGQGTLVTVSAASTKGPSVFPLAPCSRSTSESTAALGCLVKDYFPEPVTVSWNSGALTSGVHTFPAVLQSSGLYSLSSVVTVPSSSLGTKTYTCNVDHKPSNTKVDKRVESKYGPPCPPCPAPEFLGGPSVFLFPPKPKDTLMISRTPEVTCVVVDVSQEDPEVQFNWYVDGVEVHNAKTKPREEQFNSTYRVVSVLTVLHQDWLNGKEYKCKVSNKGLPSSIEKTISKAKGQPREPQVYTLPPSQEEMTKNQVSLTCLVKGFYPSDIAVEWESNGQPENNYKTTPPVLDSDGSFFLYSRLTVDKSRWQEGNVFSCSVMHEALHNHYTQKSLSLSLGK

SEQ ID NO: 10 - protein, 214 aa, synthetic construct
DILLTQSPVILSVSPGERVSFSCRASQSIGTNIHWYQQRTNGSPRLLIKYASESISGIPSRFSGSGSGTDFTLSINSVESEDIADYYCQQNNNWPTTFGAGTKLELKRTVAAPSVFIFPPSDEQLKSGTASVVCLLNNFYPREAKVQWKVDNALQSGNSQESVTEQDSKDSTYSLSSTLTLSKADYEKHKVYACEVTHQGLSSPVTKSFNRGEC

SEQ ID NO: 11 - protein, 509 aa, synthetic construct
QVQLKQSGPGLVQPSQSLSITCTVSGFSLTNYGVHWVRQSPGKGLEWLGVIWSGGNTDYNTPFTSRLSINKDNSKSQVFFKMNSLQSNDTAIYYCARALTYYDYEFAYWGQGTLVTVSAASTKGPSVFPLAPCSRSTSESTAALGCLVKDYFPEPVTVSWNSGALTSGVHTFPAVLQSSGLYSLSSVVTVPSSSLGTKTYTCNVDHKPSNTKVDKRVESKYGPPCPPCPAPEFLGGPSVFLFPPKPKDTLMISRTPEVTCVVVDVSQEDPEVQFNWYVDGVEVHNAKTKPREEQFNSTYRVVSVLTVLHQDWLNGKEYKCKVSNKGLPSSIEKTISKAKGQPREPQVYTLPPSQEEMTKNQVSLTCLVKGFYPSDIAVEWESNGQPENNYKTTPPVLDSDGSFFLYSRLTVDKSRWQEGNVFSCSVMHEALHNHYTQKSLSLSLGKGGGGSVDNKFNKEVCRAMEEIGMLPNLNAHQLAAFIWSLPDDPSQSANLLAEAKKLNDAQAPK

SEQ ID NO: 12 - protein, 214 aa, synthetic construct; identical to SEQ ID NO: 10

SEQ ID NO: 13 - protein, 572 aa, synthetic construct
QVQLKQSGPGLVQPSQSLSITCTVSGFSLTNYGVHWVRQSPGKGLEWLGVIWSGGNTDYNTPFTSRLSINKDNSKSQVFFKMNSLQSNDTAIYYCARALTYYDYEFAYWGQGTLVTVSAASTKGPSVFPLAPCSRSTSESTAALGCLVKDYFPEPVTVSWNSGALTSGVHTFPAVLQSSGLYSLSSVVTVPSSSLGTKTYTCNVDHKPSNTKVDKRVESKYGPPCPPCPAPEFLGGPSVFLFPPKPKDTLMISRTPEVTCVVVDVSQEDPEVQFNWYVDGVEVHNAKTKPREEQFNSTYRVVSVLTVLHQDWLNGKEYKCKVSNKGLPSSIEKTISKAKGQPREPQVYTLPPSQEEMTKNQVSLTCLVKGFYPSDIAVEWESNGQPENNYKTTPPVLDSDGSFFLYSRLTVDKSRWQEGNVFSCSVMHEALHNHYTQKSLSLSLGKGGGGSVDNKFNKEVCRAMEEIGMLPNLNAHQLAAFIWSLPDDPSQSANLLAEAKKLNDAQAPKGGGGSVDNKFNKEVCRAMEEIGMLPNLNAHQLAAFIWSLPDDPSQSANLLAEAKKLNDAQAPK

SEQ ID NO: 14 - protein, 214 aa, synthetic construct; identical to SEQ ID NO: 10

SEQ ID NO: 15 - protein, 509 aa, synthetic construct; identical to SEQ ID NO: 11

SEQ ID NO: 16 - protein, 277 aa, synthetic construct
DILLTQSPVILSVSPGERVSFSCRASQSIGTNIHWYQQRTNGSPRLLIKYASESISGIPSRFSGSGSGTDFTLSINSVESEDIADYYCQQNNNWPTTFGAGTKLELKRTVAAPSVFIFPPSDEQLKSGTASVVCLLNNFYPREAKVQWKVDNALQSGNSQESVTEQDSKDSTYSLSSTLTLSKADYEKHKVYACEVTHQGLSSPVTKSFNRGECGGGGSVDNKFNKEVCRAMEEIGMLPNLNAHQLAAFIWSLPDDPSQSANLLAEAKKLNDAQAPK

SEQ ID NO: 17 - protein, 446 aa, synthetic construct; identical to SEQ ID NO: 9

SEQ ID NO: 18 - protein, 340 aa, synthetic construct
DILLTQSPVILSVSPGERVSFSCRASQSIGTNIHWYQQRTNGSPRLLIKYASESISGIPSRFSGSGSGTDFTLSINSVESEDIADYYCQQNNNWPTTFGAGTKLELKRTVAAPSVFIFPPSDEQLKSGTASVVCLLNNFYPREAKVQWKVDNALQSGNSQESVTEQDSKDSTYSLSSTLTLSKADYEKHKVYACEVTHQGLSSPVTKSFNRGECGGGGSVDNKFNKEVCRAMEEIGMLPNLNAHQLAAFIWSLPDDPSQSANLLAEAKKLNDAQAPKGGGGSVDNKFNKEVCRAMEEIGMLPNLNAHQLAAFIWSLPDDPSQSANLLAEAKKLNDAQAPK

SEQ ID NO: 19 - protein, 509 aa, synthetic construct
QVQLKQSGPGLVQPSQSLSITCTVSGFSLTNYGVHWVRQSPGKGLEWLGVIWSGGNTDYNTPFTSRLSINKDNSKSQVFFKMNSLQSNDTAIYYCARALTYYDYEFAYWGQGTLVTVSAASTKGPSVFPLAPCSRSTSESTAALGCLVKDYFPEPVTVSWNSGALTSGVHTFPAVLQSSGLYSLSSVVTVPSSSLGTKTYTCNVDHKPSNTKVDKRVESKYGPPCPPCPAPEFLGGPSVFLFPPKPKDTLMISRTPEVTCVVVDVSQEDPEVQFNWYVDGVEVHNAKTKPREEQFNSTYRVVSVLTVLHQDWLNGKEYKCKVSNKGLPSSIEKTISKAKGQPREPQVYTLPPSQEEMTKNQVSLTCLVKGFYPSDIAVEWESNGQPENNYKTTPPVLDSDGSFFLYSRLTVDKSRWQEGNVFSCSVMHEALHNHYTQKSLSLSLGKGGGGSVDNKFNKEECSAMQEISMLPNLNPHQFAAFIWSLMDDPSQSANLLAEAKKLNDAQAPK

SEQ ID NO: 20 - protein, 214 aa, synthetic construct; identical to SEQ ID NO: 10

SEQ ID NO: 21 - protein, 572 aa, synthetic construct
QVQLKQSGPGLVQPSQSLSITCTVSGFSLTNYGVHWVRQSPGKGLEWLGVIWSGGNTDYNTPFTSRLSINKDNSKSQVFFKMNSLQSNDTAIYYCARALTYYDYEFAYWGQGTLVTVSAASTKGPSVFPLAPCSRSTSESTAALGCLVKDYFPEPVTVSWNSGALTSGVHTFPAVLQSSGLYSLSSVVTVPSSSLGTKTYTCNVDHKPSNTKVDKRVESKYGPPCPPCPAPEFLGGPSVFLFPPKPKDTLMISRTPEVTCVVVDVSQEDPEVQFNWYVDGVEVHNAKTKPREEQFNSTYRVVSVLTVLHQDWLNGKEYKCKVSNKGLPSSIEKTISKAKGQPREPQVYTLPPSQEEMTKNQVSLTCLVKGFYPSDIAVEWESNGQPENNYKTTPPVLDSDGSFFLYSRLTVDKSRWQEGNVFSCSVMHEALHNHYTQKSLSLSLGKGGGGSVDNKFNKEECSAMQEISMLPNLNPHQFAAFIWSLMDDPSQSANLLAEAKKLNDAQAPKGGGGSVDNKFNKEECSAMQEISMLPNLNPHQFAAFIWSLMDDPSQSANLLAEAKKLNDAQAPK

SEQ ID NO: 22 - protein, 214 aa, synthetic construct; identical to SEQ ID NO: 10

SEQ ID NO: 23 - protein, 509 aa, synthetic construct; identical to SEQ ID NO: 19

SEQ ID NO: 24 - protein, 277 aa, synthetic construct
DILLTQSPVILSVSPGERVSFSCRASQSIGTNIHWYQQRTNGSPRLLIKYASESISGIPSRFSGSGSGTDFTLSINSVESEDIADYYCQQNNNWPTTFGAGTKLELKRTVAAPSVFIFPPSDEQLKSGTASVVCLLNNFYPREAKVQWKVDNALQSGNSQESVTEQDSKDSTYSLSSTLTLSKADYEKHKVYACEVTHQGLSSPVTKSFNRGECGGGGSVDNKFNKEECSAMQEISMLPNLNPHQFAAFIWSLMDDPSQSANLLAEAKKLNDAQAPK

SEQ ID NO: 25 - protein, 446 aa, synthetic construct; identical to SEQ ID NO: 9

SEQ ID NO: 26 - protein, 340 aa, synthetic construct
DILLTQSPVILSVSPGERVSFSCRASQSIGTNIHWYQQRTNGSPRLLIKYASESISGIPSRFSGSGSGTDFTLSINSVESEDIADYYCQQNNNWPTTFGAGTKLELKRTVAAPSVFIFPPSDEQLKSGTASVVCLLNNFYPREAKVQWKVDNALQSGNSQESVTEQDSKDSTYSLSSTLTLSKADYEKHKVYACEVTHQGLSSPVTKSFNRGECGGGGSVDNKFNKEECSAMQEISMLPNLNPHQFAAFIWSLMDDPSQSANLLAEAKKLNDAQAPKGGGGSVDNKFNKEECSAMQEISMLPNLNPHQFAAFIWSLMDDPSQSANLLAEAKKLNDAQAPK

SEQ ID NO: 27 - protein, 5 aa, synthetic construct
RYWLH

SEQ ID NO: 28 - protein, 17 aa, synthetic construct
EINPSSGRTNYNEKFKS

SEQ ID NO: 29 - protein, 11 aa, synthetic construct
WDYDEGTWFAY

SEQ ID NO: 30 - protein, 11 aa, synthetic construct
RASENIYSYLA

SEQ ID NO: 31 - protein, 7 aa, synthetic construct
NARTLVE

SEQ ID NO: 32 - protein, 9 aa, synthetic construct
QHHYGPPYT

SEQ ID NO: 33 - protein, 447 aa, synthetic construct
QVQLVQSGAEVKKPGASVKVSCKASGYTFTRYWLHWVRQAPGQGLEWIGEINPSSGRTNYNEKFKSRATLTVDKSISTAYMELSRLRSDDTAVYYCARWDYDEGTWFAYWGQGTLVTVSSASTKGPSVFPLAPCSRSTSESTAALGCLVKDYFPEPVTVSWNSGALTSGVHTFPAVLQSSGLYSLSSVVTVPSSSLGTKTYTCNVDHKPSNTKVDKRVESKYGPPCPPCPAPEFLGGPSVFLFPPKPKDTLMISRTPEVTCVVVDVSQEDPEVQFNWYVDGVEVHNAKTKPREEQFNSTYRVVSVLTVLHQDWLNGKEYKCKVSNKGLPSSIEKTISKAKGQPREPQVYTLPPSQEEMTKNQVSLTCLVKGFYPSDIAVEWESNGQPENNYKTTPPVLDSDGSFFLYSRLTVDKSRWQEGNVFSCSVMHEALHNHYTQKSLSLSLGK

SEQ ID NO: 34 - protein, 214 aa, synthetic construct
DIQMTQSPSFLSASVGDRVTITCRASENIYSYLAWYQQKPGKAPKLLVYNARTLVEGVPSRFSGSGSGTEFTLTISSLQPEDFATYYCQHHYGPPYTFGQGTKVEIKRTVAAPSVFIFPPSDEQLKSGTASVVCLLNNFYPREAKVQWKVDNALQSGNSQESVTEQDSKDSTYSLSSTLTLSKADYEKHKVYACEVTHQGLSSPVTKSFNRGEC

SEQ ID NO: 35 - protein, 510 aa, synthetic construct
QVQLVQSGAEVKKPGASVKVSCKASGYTFTRYWLHWVRQAPGQGLEWIGEINPSSGRTNYNEKFKSRATLTVDKSISTAYMELSRLRSDDTAVYYCARWDYDEGTWFAYWGQGTLVTVSSASTKGPSVFPLAPCSRSTSESTAALGCLVKDYFPEPVTVSWNSGALTSGVHTFPAVLQSSGLYSLSSVVTVPSSSLGTKTYTCNVDHKPSNTKVDKRVESKYGPPCPPCPAPEFLGGPSVFLFPPKPKDTLMISRTPEVTCVVVDVSQEDPEVQFNWYVDGVEVHNAKTKPREEQFNSTYRVVSVLTVLHQDWLNGKEYKCKVSNKGLPSSIEKTISKAKGQPREPQVYTLPPSQEEMTKNQVSLTCLVKGFYPSDIAVEWESNGQPENNYKTTPPVLDSDGSFFLYSRLTVDKSRWQEGNVFSCSVMHEALHNHYTQKSLSLSLGKGGGGSVDNKFNKEVCRAMEEIGMLPNLNAHQLAAFIWSLPDDPSQSANLLAEAKKLNDAQAPK

SEQ ID NO: 36 - protein, 214 aa, synthetic construct; identical to SEQ ID NO: 34

SEQ ID NO: 37 - protein, 573 aa, synthetic construct
QVQLVQSGAEVKKPGASVKVSCKASGYTFTRYWLHWVRQAPGQGLEWIGEINPSSGRTNYNEKFKSRATLTVDKSISTAYMELSRLRSDDTAVYYCARWDYDEGTWFAYWGQGTLVTVSSASTKGPSVFPLAPCSRSTSESTAALGCLVKDYFPEPVTVSWNSGALTSGVHTFPAVLQSSGLYSLSSVVTVPSSSLGTKTYTCNVDHKPSNTKVDKRVESKYGPPCPPCPAPEFLGGPSVFLFPPKPKDTLMISRTPEVTCVVVDVSQEDPEVQFNWYVDGVEVHNAKTKPREEQFNSTYRVVSVLTVLHQDWLNGKEYKCKVSNKGLPSSIEKTISKAKGQPREPQVYTLPPSQEEMTKNQVSLTCLVKGFYPSDIAVEWESNGQPENNYKTTPPVLDSDGSFFLYSRLTVDKSRWQEGNVFSCSVMHEALHNHYTQKSLSLSLGKGGGGSVDNKFNKEVCRAMEEIGMLPNLNAHQLAAFIWSLPDDPSQSANLLAEAKKLNDAQAPKGGGGSVDNKFNKEVCRAMEEIGMLPNLNAHQLAAFIWSLPDDPSQSANLLAEAKKLNDAQAPK

SEQ ID NO: 38 - protein, 72 aa, synthetic construct
DIQMTQSPSFLSASVGDRVTITCRASENIYSYLAWYQQKPGKAPKLLVYNARTLVEGVPSRFSGSGSGTEFT

SEQ ID NO: 39 - protein, 510 aa, synthetic construct; identical to SEQ ID NO: 35

SEQ ID NO: 40 - protein, 277 aa, synthetic construct
DIQMTQSPSFLSASVGDRVTITCRASENIYSYLAWYQQKPGKAPKLLVYNARTLVEGVPSRFSGSGSGTEFTLTISSLQPEDFATYYCQHHYGPPYTFGQGTKVEIKRTVAAPSVFIFPPSDEQLKSGTASVVCLLNNFYPREAKVQWKVDNALQSGNSQESVTEQDSKDSTYSLSSTLTLSKADYEKHKVYACEVTHQGLSSPVTKSFNRGECGGGGSVDNKFNKEVCRAMEEIGMLPNLNAHQLAAFIWSLPDDPSQSANLLAEAKKLNDAQAPK

SEQ ID NO: 41 - protein, 447 aa, synthetic construct; identical to SEQ ID NO: 33

SEQ ID NO: 42 - protein, 340 aa, synthetic construct
DIQMTQSPSFLSASVGDRVTITCRASENIYSYLAWYQQKPGKAPKLLVYNARTLVEGVPSRFSGSGSGTEFTLTISSLQPEDFATYYCQHHYGPPYTFGQGTKVEIKRTVAAPSVFIFPPSDEQLKSGTASVVCLLNNFYPREAKVQWKVDNALQSGNSQESVTEQDSKDSTYSLSSTLTLSKADYEKHKVYACEVTHQGLSSPVTKSFNRGECGGGGSVDNKFNKEVCRAMEEIGMLPNLNAHQLAAFIWSLPDDPSQSANLLAEAKKLNDAQAPKGGGGSVDNKFNKEVCRAMEEIGMLPNLNAHQLAAFIWSLPDDPSQSANLLAEAKKLNDAQAPK

SEQ ID NO: 43 - protein, 510 aa, synthetic construct
QVQLVQSGAEVKKPGASVKVSCKASGYTFTRYWLHWVRQAPGQGLEWIGEINPSSGRTNYNEKFKSRATLTVDKSISTAYMELSRLRSDDTAVYYCARWDYDEGTWFAYWGQGTLVTVSSASTKGPSVFPLAPCSRSTSESTAALGCLVKDYFPEPVTVSWNSGALTSGVHTFPAVLQSSGLYSLSSVVTVPSSSLGTKTYTCNVDHKPSNTKVDKRVESKYGPPCPPCPAPEFLGGPSVFLFPPKPKDTLMISRTPEVTCVVVDVSQEDPEVQFNWYVDGVEVHNAKTKPREEQFNSTYRVVSVLTVLHQDWLNGKEYKCKVSNKGLPSSIEKTISKAKGQPREPQVYTLPPSQEEMTKNQVSLTCLVKGFYPSDIAVEWESNGQPENNYKTTPPVLDSDGSFFLYSRLTVDKSRWQEGNVFSCSVMHEALHNHYTQKSLSLSLGKGGGGSVDNKFNKEECSAMQEISMLPNLNPHQFAAFIWSLMDDPSQSANLLAEAKKLNDAQAPK

SEQ ID NO: 44 - protein, 214 aa, synthetic construct; identical to SEQ ID NO: 34

SEQ ID NO: 45 - protein, 573 aa, synthetic construct
QVQLVQSGAEVKKPGASVKVSCKASGYTFTRYWLHWVRQAPGQGLEWIGEINPSSGRTNYNEKFKSRATLTVDKSISTAYMELSRLRSDDTAVYYCARWDYDEGTWFAYWGQGTLVTVSSASTKGPSVFPLAPCSRSTSESTAALGCLVKDYFPEPVTVSWNSGALTSGVHTFPAVLQSSGLYSLSSVVTVPSSSLGTKTYTCNVDHKPSNTKVDKRVESKYGPPCPPCPAPEFLGGPSVFLFPPKPKDTLMISRTPEVTCVVVDVSQEDPEVQFNWYVDGVEVHNAKTKPREEQFNSTYRVVSVLTVLHQDWLNGKEYKCKVSNKGLPSSIEKTISKAKGQPREPQVYTLPPSQEEMTKNQVSLTCLVKGFYPSDIAVEWESNGQPENNYKTTPPVLDSDGSFFLYSRLTVDKSRWQEGNVFSCSVMHEALHNHYTQKSLSLSLGKGGGGSVDNKFNKEECSAMQEISMLPNLNPHQFAAFIWSLMDDPSQSANLLAEAKKLNDAQAPKGGGGSVDNKFNKEECSAMQEISMLPNLNPHQFAAFIWSLMDDPSQSANLLAEAKKLNDAQAPK

SEQ ID NO: 46 - protein, 214 aa, synthetic construct; identical to SEQ ID NO: 34

SEQ ID NO: 47 - protein, 510 aa, synthetic construct; identical to SEQ ID NO: 43

SEQ ID NO: 48 - protein, 277 aa, synthetic construct
DIQMTQSPSFLSASVGDRVTITCRASENIYSYLAWYQQKPGKAPKLLVYNARTLVEGVPSRFSGSGSGTEFTLTISSLQPEDFATYYCQHHYGPPYTFGQGTKVEIKRTVAAPSVFIFPPSDEQLKSGTASVVCLLNNFYPREAKVQWKVDNALQSGNSQESVTEQDSKDSTYSLSSTLTLSKADYEKHKVYACEVTHQGLSSPVTKSFNRGECGGGGSVDNKFNKEECSAMQEISMLPNLNPHQFAAFIWSLMDDPSQSANLLAEAKKLNDAQAPK

SEQ ID NO: 49 - protein, 447 aa, synthetic construct; identical to SEQ ID NO: 33

SEQ ID NO: 50 - protein, 340 aa, synthetic construct
DIQMTQSPSFLSASVGDRVTITCRASENIYSYLAWYQQKPGKAPKLLVYNARTLVEGVPSRFSGSGSGTEFTLTISSLQPEDFATYYCQHHYGPPYTFGQGTKVEIKRTVAAPSVFIFPPSDEQLKSGTASVVCLLNNFYPREAKVQWKVDNALQSGNSQESVTEQDSKDSTYSLSSTLTLSKADYEKHKVYACEVTHQGLSSPVTKSFNRGECGGGGSVDNKFNKEECSAMQEISMLPNLNPHQFAAFIWSLMDDPSQSANLLAEAKKLNDAQAPKGGGGSVDNKFNKEECSAMQEISMLPNLNPHQFAAFIWSLMDDPSQSANLLAEAKKLNDAQAPK

SEQ ID NO: 51 - protein, 5 aa, synthetic construct
EYTIH

SEQ ID NO: 52 - protein, 17 aa, synthetic construct
NINPNNGGTTYNQKFED

SEQ ID NO: 53 - protein, 6 aa, synthetic construct
GWNFDY

SEQ ID NO: 54 - protein, 11 aa, synthetic construct
KASQDVGTAVD

SEQ ID NO: 55 - protein, 7 aa, synthetic construct
WASTRHT

SEQ ID NO: 56 - protein, 9 aa, synthetic construct
QQYNSYPLT

SEQ ID NO: 57 - protein, 442 aa, synthetic construct
EVQLVQSGPEVKKPGATVKISCKTSGYTFTEYTIHWVKQAPGKGLEWIGNINPNNGGTTYNQKFEDKATLTVDKSTDTAYMELSSLRSEDTAVYYCAAGWNFDYWGQGTLLTVSSASTKGPSVFPLAPCSRSTSESTAALGCLVKDYFPEPVTVSWNSGALTSGVHTFPAVLQSSGLYSLSSVVTVPSSSLGTKTYTCNVDHKPSNTKVDKRVESKYGPPCPPCPAPEFLGGPSVFLFPPKPKDTLMISRTPEVTCVVVDVSQEDPEVQFNWYVDGVEVHNAKTKPREEQFNSTYRVVSVLTVLHQDWLNGKEYKCKVSNKGLPSSIEKTISKAKGQPREPQVYTLPPSQEEMTKNQVSLTCLVKGFYPSDIAVEWESNGQPENNYKTTPPVLDSDGSFFLYSRLTVDKSRWQEGNVFSCSVMHEALHNHYTQKSLSLSLGK

SEQ ID NO: 58 - protein, 214 aa, synthetic construct
DIQMTQSPSSLSTSVGDRVTLTCKASQDVGTAVDWYQQKPGPSPKLLIYWASTRHTGIPSRFSGSGSGTDFTLTISSLQPEDFADYYCQQYNSYPLTFGPGTKVDIKRTVAAPSVFIFPPSDEQLKSGTASVVCLLNNFYPREAKVQWKVDNALQSGNSQESVTEQDSKDSTYSLSSTLTLSKADYEKHKVYACEVTHQGLSSPVTKSFNRGEC

SEQ ID NO: 59 - protein, 505 aa, synthetic construct
EVQLVQSGPEVKKPGATVKISCKTSGYTFTEYTIHWVKQAPGKGLEWIGNINPNNGGTTYNQKFEDKATLTVDKSTDTAYMELSSLRSEDTAVYYCAAGWNFDYWGQGTLLTVSSASTKGPSVFPLAPCSRSTSESTAALGCLVKDYFPEPVTVSWNSGALTSGVHTFPAVLQSSGLYSLSSVVTVPSSSLGTKTYTCNVDHKPSNTKVDKRVESKYGPPCPPCPAPEFLGGPSVFLFPPKPKDTLMISRTPEVTCVVVDVSQEDPEVQFNWYVDGVEVHNAKTKPREEQFNSTYRVVSVLTVLHQDWLNGKEYKCKVSNKGLPSSIEKTISKAKGQPREPQVYTLPPSQEEMTKNQVSLTCLVKGFYPSDIAVEWESNGQPENNYKTTPPVLDSDGSFFLYSRLTVDKSRWQEGNVFSCSVMHEALHNHYTQKSLSLSLGKGGGGSVDNKFNKEVCRAMEEIGMLPNLNAHQLAAFIWSLPDDPSQSANLLAEAKKLNDAQAPK

SEQ ID NO: 60 - protein, 214 aa, synthetic construct; identical to SEQ ID NO: 58

SEQ ID NO: 61 - protein, 568 aa, synthetic construct
EVQLVQSGPEVKKPGATVKISCKTSGYTFTEYTIHWVKQAPGKGLEWIGNINPNNGGTTYNQKFEDKATLTVDKSTDTAYMELSSLRSEDTAVYYCAAGWNFDYWGQGTLLTVSSASTKGPSVFPLAPCSRSTSESTAALGCLVKDYFPEPVTVSWNSGALTSGVHTFPAVLQSSGLYSLSSVVTVPSSSLGTKTYTCNVDHKPSNTKVDKRVESKYGPPCPPCPAPEFLGGPSVFLFPPKPKDTLMISRTPEVTCVVVDVSQEDPEVQFNWYVDGVEVHNAKTKPREEQFNSTYRVVSVLTVLHQDWLNGKEYKCKVSNKGLPSSIEKTISKAKGQPREPQVYTLPPSQEEMTKNQVSLTCLVKGFYPSDIAVEWESNGQPENNYKTTPPVLDSDGSFFLYSRLTVDKSRWQEGNVFSCSVMHEALHNHYTQKSLSLSLGKGGGGSVDNKFNKEVCRAMEEIGMLPNLNAHQLAAFIWSLPDDPSQSANLLAEAKKLNDAQAPKGGGGSVDNKFNKEVCRAMEEIGMLPNLNAHQLAAFIWSLPDDPSQSANLLAEAKKLNDAQAPK

SEQ ID NO: 62 - protein, 214 aa, synthetic construct; identical to SEQ ID NO: 58

SEQ ID NO: 63 - protein, 505 aa, synthetic construct; identical to SEQ ID NO: 59

SEQ ID NO: 64 - protein, 277 aa, synthetic construct
DIQMTQSPSSLSTSVGDRVTLTCKASQDVGTAVDWYQQKPGPSPKLLIYWASTRHTGIPSRFSGSGSGTDFTLTISSLQPEDFADYYCQQYNSYPLTFGPGTKVDIKRTVAAPSVFIFPPSDEQLKSGTASVVCLLNNFYPREAKVQWKVDNALQSGNSQESVTEQDSKDSTYSLSSTLTLSKADYEKHKVYACEVTHQGLSSPVTKSFNRGECGGGGSVDNKFNKEVCRAMEEIGMLPNLNAHQLAAFIWSLPDDPSQSANLLAEAKKLNDAQAPK

SEQ ID NO: 65 - protein, 442 aa, synthetic construct; identical to SEQ ID NO: 57

SEQ ID NO: 66 - protein, 339 aa, synthetic construct
DIQMTQSPSSLSTSVGDRVTLTCKASQDVGTAVDWYQQKPGPSPKLLIYWASTRHTGIPSRFSGSGSGTDFTLTISSLQPEDFADYYCQQYNSYPLTFGPGTKVDIKRTVAAPSVFIFPPSDEQLKSGTASVVCLLNNFYPREAKVQWKVDNALQSGNSQESVTEQDSKDSTYSLSSTLTLSKADYEKHKVYACEVTHQGLSSPVTKSFNRGECGGGGSVDNKFNKEVCRAMEEIGMLPNLNAHQLAAFIWSLPDDPSQSANLLAEAKKLNDAQAPKGGGSVDNKFNKEVCRAMEEIGMLPNLNAHQLAAFIWSLPDDPSQSANLLAEAKKLNDAQAPK

SEQ ID NO: 67 - protein, 505 aa, synthetic construct
EVQLVQSGPEVKKPGATVKISCKTSGYTFTEYTIHWVKQAPGKGLEWIGNINPNNGGTTYNQKFEDKATLTVDKSTDTAYMELSSLRSEDTAVYYCAAGWNFDYWGQGTLLTVSSASTKGPSVFPLAPCSRSTSESTAALGCLVKDYFPEPVTVSWNSGALTSGVHTFPAVLQSSGLYSLSSVVTVPSSSLGTKTYTCNVDHKPSNTKVDKRVESKYGPPCPPCPAPEFLGGPSVFLFPPKPKDTLMISRTPEVTCVVVDVSQEDPEVQFNWYVDGVEVHNAKTKPREEQFNSTYRVVSVLTVLHQDWLNGKEYKCKVSNKGLPSSIEKTISKAKGQPREPQVYTLPPSQEEMTKNQVSLTCLVKGFYPSDIAVEWESNGQPENNYKTTPPVLDSDGSFFLYSRLTVDKSRWQEGNVFSCSVMHEALHNHYTQKSLSLSLGKGGGGSVDNKFNKEECSAMQEISMLPNLNPHQFAAFIWSLMDDPSQSANLLAEAKKLNDAQAPK

SEQ ID NO: 68 - protein, 214 aa, synthetic construct; identical to SEQ ID NO: 58

SEQ ID NO: 69 - protein, 568 aa, synthetic construct
EVQLVQSGPEVKKPGATVKISCKTSGYTFTEYTIHWVKQAPGKGLEWIGNINPNNGGTTYNQKFEDKATLTVDKSTDTAYMELSSLRSEDTAVYYCAAGWNFDYWGQGTLLTVSSASTKGPSVFPLAPCSRSTSESTAALGCLVKDYFPEPVTVSWNSGALTSGVHTFPAVLQSSGLYSLSSVVTVPSSSLGTKTYTCNVDHKPSNTKVDKRVESKYGPPCPPCPAPEFLGGPSVFLFPPKPKDTLMISRTPEVTCVVVDVSQEDPEVQFNWYVDGVEVHNAKTKPREEQFNSTYRVVSVLTVLHQDWLNGKEYKCKVSNKGLPSSIEKTISKAKGQPREPQVYTLPPSQEEMTKNQVSLTCLVKGFYPSDIAVEWESNGQPENNYKTTPPVLDSDGSFFLYSRLTVDKSRWQEGNVFSCSVMHEALHNHYTQKSLSLSLGKGGGGSVDNKFNKEECSAMQEISMLPNLNPHQFAAFIWSLMDDPSQSANLLAEAKKLNDAQAPKGGGGSVDNKFNKEECSAMQEISMLPNLNPHQFAAFIWSLMDDPSQSANLLAEAKKLNDAQAPK

SEQ ID NO: 70 - protein, 214 aa, synthetic construct; identical to SEQ ID NO: 58

SEQ ID NO: 71 - protein, 505 aa, synthetic construct; identical to SEQ ID NO: 67

SEQ ID NO: 72 - protein, 277 aa, synthetic construct
DIQMTQSPSSLSTSVGDRVTLTCKASQDVGTAVDWYQQKPGPSPKLLIYWASTRHTGIPSRFSGSGSGTDFTLTISSLQPEDFADYYCQQYNSYPLTFGPGTKVDIKRTVAAPSVFIFPPSDEQLKSGTASVVCLLNNFYPREAKVQWKVDNALQSGNSQESVTEQDSKDSTYSLSSTLTLSKADYEKHKVYACEVTHQGLSSPVTKSFNRGECGGGGSVDNKFNKEECSAMQEISMLPNLNPHQFAAFIWSLMDDPSQSANLLAEAKKLNDAQAPK

SEQ ID NO: 73 - protein, 442 aa, synthetic construct; identical to SEQ ID NO: 57

SEQ ID NO: 74 - protein, 340 aa, synthetic construct
DIQMTQSPSSLSTSVGDRVTLTCKASQDVGTAVDWYQQKPGPSPKLLIYWASTRHTGIPSRFSGSGSGTDFTLTISSLQPEDFADYYCQQYNSYPLTFGPGTKVDIKRTVAAPSVFIFPPSDEQLKSGTASVVCLLNNFYPREAKVQWKVDNALQSGNSQESVTEQDSKDSTYSLSSTLTLSKADYEKHKVYACEVTHQGLSSPVTKSFNRGECGGGGSVDNKFNKEECSAMQEISMLPNLNPHQFAAFIWSLMDDPSQSANLLAEAKKLNDAQAPKGGGGSVDNKFNKEECSAMQEISMLPNLNPHQFAAFIWSLMDDPSQSANLLAEAKKLNDAQAPK

SEQ ID NO: 75 - DNA, 174 bp, synthetic construct
  source 1..174: mol_type = other DNA
gtggataacaaatttaacaaagaggtgtgcagagctatggaggaaataggaatgctgcccaacttaaacgcccaccaactggccgctttcatctggtcactgccagacgatcccagccagagcgccaatctgcttgctgaggccaaaaagctgaacgacgcccaggcccctaag

SEQ ID NO: 76 - DNA, 174 bp, synthetic construct
  source 1..174: mol_type = other DNA
gtggacaacaagttcaacaaggaggaatgctctgccatgcaggagatttctatgctgcccaacctgaacccgcatcagttcgctgccttcatttggtccctgatggacgacccttcccagtccgccaacctgctggccgaggccaagaagctgaacgacgcccaggctcccaag

SEQ ID NO: 77 - DNA, 15 bp, synthetic construct
  source 1..15: mol_type = other DNA
aattatggcgtgcac

SEQ ID NO: 78 - DNA, 48 bp, synthetic construct
  source 1..48: mol_type = other DNA
gtgatttggagcggcgggaacaccgactataataccccattcaccagc

SEQ ID NO: 79 - DNA, 33 bp, synthetic construct
  source 1..33: mol_type = other DNA
gctctgacctattatgattatgagttcgcttac

SEQ ID NO: 80 - DNA, 33 bp, synthetic construct
  source 1..33: mol_type = other DNA
agggcctcgcaaagcatagggacgaatatccac

SEQ ID NO: 81 - DNA, 21 bp, synthetic construct
  source 1..21: mol_type = other DNA
tacgcttctgaatccatatct

SEQ ID NO: 82 - DNA, 27 bp, synthetic construct
  source 1..27: mol_type = other DNA
cagcaaaataacaactggccaaccacc

SEQ ID NO: 83 - DNA, 1338 bp, synthetic construct
  source 1..1338: mol_type = other DNA
caggtgcagttgaagcagagcggccccggcctggttcagcccagccaatcactgagcatcacttgcaccgtaagcggctttagcttgaccaattatggcgtgcactgggtgagacaaagccctggcaaggggctggagtggctgggagtgatttggagcggcgggaacaccgactataataccccattcaccagcagactgagcattaataaggacaatagcaaatcgcaggtgttctttaaaatgaatagccttcagagcaacgacaccgcgatatactactgtgcaagagctctgacctattatgattatgagttcgcttactgggggcagggtaccctggttacagtgagcgcagcatcaaccaagggacccagcgtgtttcccctggctccctgcagcagaagtaccagcgagagcaccgcggccctgggctgccttgtgaaagactactttcctgagccggtgaccgtgtcatggaattcgggcgccctgactagcggagtacacaccttcccggccgtactgcagagcagcggcctgtacagcctgagctccgtggtgacggtgcccagctctagcctaggtacgaagacctacacttgtaacgtggatcataagcccagcaacaccaaggttgacaagcgggtggaaagcaagtatggcccgccatgtccaccatgccccgcacctgagtttctggggggcccaagcgtattcctttttcccccaaaacctaaagataccctgatgatttcccgtactcccgaggtgacgtgtgtggtggtggatgtgagccaggaggatccagaggtccagttcaactggtatgtggacggcgtggaagtgcataatgcaaaaaccaaacccagagaagagcaattcaacagcacatacagggttgtgtcagttctcacagtgctgcaccaagactggctgaatggcaaggaatacaaatgtaaagttagcaataagggcctgccttcaagcatcgaaaagaccatcagcaaagccaaaggtcagccaagagaaccccaggtatacactttgcctccaagccaggaagagatgaccaaaaatcaggtgagcctgacctgcctggttaagggtttttacccgagcgatattgccgtggagtgggaaagcaatggccagcctgaaaacaattataagacaaccccccccgttctggactccgacggatcttttttcctatacagcagactgaccgtggataagtccaggtggcaggagggaaacgtgttcagctgttctgtgatgcatgaagccttacacaaccactatacccaaaagagcttatccctaagcctgggcaaa

SEQ ID NO: 84 - DNA, 642 bp, synthetic construct
  source 1..642: mol_type = other DNA
gatatcctgcttacacagagcccggtgattctgtcagtgagccctggcgaacgggtgagctttagttgcagggcctcgcaaagcatagggacgaatatccactggtatcagcagaggacaaatggctcacctcgactgttgattaaatacgcttctgaatccatatctggaattcctagtcgcttctcagggagcggctcaggtactgacttcacactgagcattaatagcgtcgagagcgaggatatcgcagattactattgccagcaaaataacaactggccaaccaccttcggagccggcaccaaactagagctgaaaagaactgtggcagcacccagcgtctttatcttccccccaagcgacgagcagctgaaatccgggacggcgtctgttgtgtgcctgctgaacaacttttatccccgggaggccaaggtgcagtggaaagtggacaacgccctgcagtcgggaaatagccaggagtccgtcaccgaacaagatagcaaggacagcacatactccctgagcagcactctgaccctgagtaaggccgactacgaaaagcacaaggtatatgcttgtgaagtcacccaccagggcctgagtagcccagttactaagtcattcaacagaggtgagtgt

SEQ ID NO: 85 - DNA, 1527 bp, synthetic construct
  source 1..1527: mol_type = other DNA
caggtgcagttgaagcagagcggccccggcctggttcagcccagccaatcactgagcatcacttgcaccgtaagcggctttagcttgaccaattatggcgtgcactgggtgagacaaagccctggcaaggggctggagtggctgggagtgatttggagcggcgggaacaccgactataataccccattcaccagcagactgagcattaataaggacaatagcaaatcgcaggtgttctttaaaatgaatagccttcagagcaacgacaccgcgatatactactgtgcaagagctctgacctattatgattatgagttcgcttactgggggcagggtaccctggttacagtgagcgcagcatcaaccaagggacccagcgtgtttcccctggctccctgcagcagaagtaccagcgagagcaccgcggccctgggctgccttgtgaaagactactttcctgagccggtgaccgtgtcatggaattcgggcgccctgactagcggagtacacaccttcccggccgtactgcagagcagcggcctgtacagcctgagctccgtggtgacggtgcccagctctagcctaggtacgaagacctacacttgtaacgtggatcataagcccagcaacaccaaggttgacaagcgggtggaaagcaagtatggcccgccatgtccaccatgccccgcacctgagtttctggggggcccaagcgtattcctttttcccccaaaacctaaagataccctgatgatttcccgtactcccgaggtgacgtgtgtggtggtggatgtgagccaggaggatccagaggtccagttcaactggtatgtggacggcgtggaagtgcataatgcaaaaaccaaacccagagaagagcaattcaacagcacatacagggttgtgtcagttctcacagtgctgcaccaagactggctgaatggcaaggaatacaaatgtaaagttagcaataagggcctgccttcaagcatcgaaaagaccatcagcaaagccaaaggtcagccaagagaaccccaggtatacactttgcctccaagccaggaagagatgaccaaaaatcaggtgagcctgacctgcctggttaagggtttttacccgagcgatattgccgtggagtgggaaagcaatggccagcctgaaaacaattataagacaaccccccccgttctggactccgacggatcttttttcctatacagcagactgaccgtggataagtccaggtggcaggagggaaacgtgttcagctgttctgtgatgcatgaagccttacacaaccactatacccaaaagagcttatccctaagcctgggcaaagggggcggcggaagcgtggataacaaatttaacaaagaggtgtgcagagctatggaggaaataggaatgctgcccaacttaaacgcccaccaactggccgctttcatctggtcactgccagacgatcccagccagagcgccaatctgcttgctgaggccaaaaagctgaacgacgcccaggcccctaag

SEQ ID NO: 86 - DNA, 642 bp, synthetic construct; identical to SEQ ID NO: 84
  source 1..642: mol_type = other DNA

SEQ ID NO: 87 - DNA, 1716 bp, synthetic construct
  source 1..1716: mol_type = other DNA
caggtgcagttgaagcagagcggccccggcctggttcagcccagccaatcactgagcatcacttgcaccgtaagcggctttagcttgaccaattatggcgtgcactgggtgagacaaagccctggcaaggggctggagtggctgggagtgatttggagcggcgggaacaccgactataataccccattcaccagcagactgagcattaataaggacaatagcaaatcgcaggtgttctttaaaatgaatagccttcagagcaacgacaccgcgatatactactgtgcaagagctctgacctattatgattatgagttcgcttactgggggcagggtaccctggttacagtgagcgcagcatcaaccaagggacccagcgtgtttcccctggctccctgcagcagaagtaccagcgagagcaccgcggccctgggctgccttgtgaaagactactttcctgagccggtgaccgtgtcatggaattcgggcgccctgactagcggagtacacaccttcccggccgtactgcagagcagcggcctgtacagcctgagctccgtggtgacggtgcccagctctagcctaggtacgaagacctacacttgtaacgtggatcataagcccagcaacaccaaggttgacaagcgggtggaaagcaagtatggcccgccatgtccaccatgccccgcacctgagtttctggggggcccaagcgtattcctttttcccccaaaacctaaagataccctgatgatttcccgtactcccgaggtgacgtgtgtggtggtggatgtgagccaggaggatccagaggtccagttcaactggtatgtggacggcgtggaagtgcataatgcaaaaaccaaacccagagaagagcaattcaacagcacatacagggttgtgtcagttctcacagtgctgcaccaagactggctgaatggcaaggaatacaaatgtaaagttagcaataagggcctgccttcaagcatcgaaaagaccatcagcaaagccaaaggtcagccaagagaaccccaggtatacactttgcctccaagccaggaagagatgaccaaaaatcaggtgagcctgacctgcctggttaagggtttttacccgagcgatattgccgtggagtgggaaagcaatggccagcctgaaaacaattataagacaaccccccccgttctggactccgacggatcttttttcctatacagcagactgaccgtggataagtccaggtggcaggagggaaacgtgttcagctgttctgtgatgcatgaagccttacacaaccactatacccaaaagagcttatccctaagcctgggcaaaggtggaggtggaagcgtggataacaaatttaacaaagaggtgtgcagagctatggaggaaataggaatgctgcccaacttaaacgcccaccaactggccgctttcatctggtcactgccagacgatcccagccagagcgccaatctgcttgctgaggccaaaaagctgaatgacgcccaggcccctaaggggggcggcggaagcgtggataacaaatttaacaaagaggtgtgcagagctatggaggaaataggaatgctgcccaacttaaacgcccaccaactggccgctttcatctggtcactgccagacgatcccagccagagcgccaatctgcttgctgaggccaaaaagctgaacgacgcccaggcccctaag

SEQ ID NO: 88 - DNA, 642 bp, synthetic construct; identical to SEQ ID NO: 84
  source 1..642: mol_type = other DNA

SEQ ID NO: 89 - DNA, 1527 bp, synthetic construct; identical to SEQ ID NO: 85
  source 1..1527: mol_type = other DNA

SEQ ID NO: 90 - DNA, 831 bp, synthetic construct
  source 1..831: mol_type = other DNA
gatatcctgcttacacagagcccggtgattctgtcagtgagccctggcgaacgggtgagctttagttgcagggcctcgcaaagcatagggacgaatatccactggtatcagcagaggacaaatggctcacctcgactgttgattaaatacgcttctgaatccatatctggaattcctagtcgcttctcagggagcggctcaggtactgacttcacactgagcattaatagcgtcgagagcgaggatatcgcagattactattgccagcaaaataacaactggccaaccaccttcggagccggcaccaaactagagctgaaaagaactgtggcagcacccagcgtctttatcttccccccaagcgacgagcagctgaaatccgggacggcgtctgttgtgtgcctgctgaacaacttttatccccgggaggccaaggtgcagtggaaagtggacaacgccctgcagtcgggaaatagccaggagtccgtcaccgaacaagatagcaaggacagcacatactccctgagcagcactctgaccctgagtaaggccgactacgaaaagcacaaggtatatgcttgtgaagtcacccaccagggcctgagtagcccagttactaagtcattcaacagaggtgaatgtgggggcggcggaagcgtggacaacaagttcaacaaggaggtttgccgtgccatggaagagattggtatgctgcccaacctgaacgctcatcagctggctgccttcatttggtccctgccggacgacccttcccagtccgccaacctgctggccgaggccaagaagctgaacgacgcccaggctcccaag

SEQ ID NO: 91 - DNA, 1338 bp, synthetic construct; identical to SEQ ID NO: 83
  source 1..1338: mol_type = other DNA

SEQ ID NO: 92 - DNA, 1020 bp, synthetic construct
  source 1..1020: mol_type = other DNA
gatatcctgcttacacagagcccggtgattctgtcagtgagccctggcgaacgggtgagctttagttgcagggcctcgcaaagcatagggacgaatatccactggtatcagcagaggacaaatggctcacctcgactgttgattaaatacgcttctgaatccatatctggaattcctagtcgcttctcagggagcggctcaggtactgacttcacactgagcattaatagcgtcgagagcgaggatatcgcagattactattgccagcaaaataacaactggccaaccaccttcggagccggcaccaaactagagctgaaaagaactgtggcagcacccagcgtctttatcttccccccaagcgacgagcagctgaaatccgggacggcgtctgttgtgtgcctgctgaacaacttttatccccgggaggccaaggtgcagtggaaagtggacaacgccctgcagtcgggaaatagccaggagtccgtcaccgaacaagatagcaaggacagcacatactccctgagcagcactctgaccctgagtaaggccgactacgaaaagcacaaggtatatgcttgtgaagtcacccaccagggcctgagtagcccagttactaagtcattcaacagaggtgagtgtggtggaggtggaagcgtggataacaaatttaacaaagaggtgtgcagagctatggaggaaataggaatgctgcccaacttaaacgcccaccaactggccgctttcatctggtcactgccagacgatcccagccagagcgccaatctgcttgctgaggccaaaaagctgaatgacgcccaggcccctaaggggggcggcggaagcgtggataacaaatttaacaaagaggtgtgcagagctatggaggaaataggaatgctgcccaacttaaacgcccaccaactggccgctttcatctggtcactgccagacgatcccagccagagcgccaatctgcttgctgaggccaaaaagctgaacgacgcccaggcccctaag

SEQ ID NO: 93 - DNA, 1527 bp, synthetic construct
  source 1..1527: mol_type = other DNA
caggtgcagttgaagcagagcggccccggcctggttcagcccagccaatcactgagcatcacttgcaccgtaagcggctttagcttgaccaattatggcgtgcactgggtgagacaaagccctggcaaggggctggagtggctgggagtgatttggagcggcgggaacaccgactataataccccattcaccagcagactgagcattaataaggacaatagcaaatcgcaggtgttctttaaaatgaatagccttcagagcaacgacaccgcgatatactactgtgcaagagctctgacctattatgattatgagttcgcttactgggggcagggtaccctggttacagtgagcgcagcatcaaccaagggacccagcgtgtttcccctggctccctgcagcagaagtaccagcgagagcaccgcggccctgggctgccttgtgaaagactactttcctgagccggtgaccgtgtcatggaattcgggcgccctgactagcggagtacacaccttcccggccgtactgcagagcagcggcctgtacagcctgagctccgtggtgacggtgcccagctctagcctaggtacgaagacctacacttgtaacgtggatcataagcccagcaacaccaaggttgacaagcgggtggaaagcaagtatggcccgccatgtccaccatgccccgcacctgagtttctggggggcccaagcgtattcctttttcccccaaaacctaaagataccctgatgatttcccgtactcccgaggtgacgtgtgtggtggtggatgtgagccaggaggatccagaggtccagttcaactggtatgtggacggcgtggaagtgcataatgcaaaaaccaaacccagagaagagcaattcaacagcacatacagggttgtgtcagttctcacagtgctgcaccaagactggctgaatggcaaggaatacaaatgtaaagttagcaataagggcctgccttcaagcatcgaaaagaccatcagcaaagccaaaggtcagccaagagaaccccaggtatacactttgcctccaagccaggaagagatgaccaaaaatcaggtgagcctgacctgcctggttaagggtttttacccgagcgatattgccgtggagtgggaaagcaatggccagcctgaaaacaattataagacaaccccccccgttctggactccgacggatcttttttcctatacagcagactgaccgtggataagtccaggtggcaggagggaaacgtgttcagctgttctgtgatgcatgaagccttacacaaccactatacccaaaagagcttatccctaagcctgggcaaagggggcggcggaagcgtggacaacaagttcaacaaggaggaatgctctgccatgcaggagatttctatgctgcccaacctgaacccgcatcagttcgctgccttcatttggtccctgatggacgacccttcccagtccgccaacctgctggccgaggccaagaagctgaacgacgcccaggctcccaag

SEQ ID NO: 94 - DNA, 642 bp, synthetic construct; identical to SEQ ID NO: 84
  source 1..642: mol_type = other DNA

SEQ ID NO: 95 - DNA, 1716 bp, synthetic construct
  source 1..1716: mol_type = other DNA
caggtgcagttgaagcagagcggccccggcctggttcagcccagccaatcactgagcatcacttgcaccgtaagcggctttagcttgaccaattatggcgtgcactgggtgagacaaagccctggcaaggggctggagtggctgggagtgatttggagcggcgggaacaccgactataataccccattcaccagcagactgagcattaataaggacaatagcaaatcgcaggtgttctttaaaatgaatagccttcagagcaacgacaccgcgatatactactgtgcaagagctctgacctattatgattatgagttcgcttactgggggcagggtaccctggttacagtgagcgcagcatcaaccaagggacccagcgtgtttcccctggctccctgcagcagaagtaccagcgagagcaccgcggccctgggctgccttgtgaaagactactttcctgagccggtgaccgtgtcatggaattcgggcgccctgactagcggagtacacaccttcccggccgtactgcagagcagcggcctgtacagcctgagctccgtggtgacggtgcccagctctagcctaggtacgaagacctacacttgtaacgtggatcataagcccagcaacaccaaggttgacaagcgggtggaaagcaagtatggcccgccatgtccaccatgccccgcacctgagtttctggggggcccaagcgtattcctttttcccccaaaacctaaagataccctgatgatttcccgtactcccgaggtgacgtgtgtggtggtggatgtgagccaggaggatccagaggtccagttcaactggtatgtggacggcgtggaagtgcataatgcaaaaaccaaacccagagaagagcaattcaacagcacatacagggttgtgtcagttctcacagtgctgcaccaagactggctgaatggcaaggaatacaaatgtaaagttagcaataagggcctgccttcaagcatcgaaaagaccatcagcaaagccaaaggtcagccaagagaaccccaggtatacactttgcctccaagccaggaagagatgaccaaaaatcaggtgagcctgacctgcctggttaagggtttttacccgagcgatattgccgtggagtgggaaagcaatggccagcctgaaaacaattataagacaaccccccccgttctggactccgacggatcttttttcctatacagcagactgaccgtggataagtccaggtggcaggagggaaacgtgttcagctgttctgtgatgcatgaagccttacacaaccactatacccaaaagagcttatccctaagcctgggcaaaggtggaggtggaagcgtggacaacaagttcaacaaggaggaatgctctgccatgcaggagatttctatgctgcccaacctgaacccgcatcagttcgctgccttcatttggtccctgatggacgacccttcccagtccgccaacctgctggccgaggccaagaagctgaacgacgcccaggctcccaaggggggcggcggaagcgtggacaacaagttcaacaaggaggaatgctctgccatgcaggagatttctatgctgcccaacctgaacccgcatcagttcgctgccttcatttggtccctgatggacgacccttcccagtccgccaacctgctggccgaggccaagaagctgaacgacgcccaggctcccaag

SEQ ID NO: 96 - DNA, 642 bp, synthetic construct; identical to SEQ ID NO: 84
  source 1..642: mol_type = other DNA

SEQ ID NO: 97 - DNA, 1527 bp, synthetic construct; identical to SEQ ID NO: 93
  source 1..1527: mol_type = other DNA

SEQ ID NO: 98 - DNA, 831 bp, synthetic construct
  source 1..831: mol_type = other DNA
gatatcctgcttacacagagcccggtgattctgtcagtgagccctggcgaacgggtgagctttagttgcagggcctcgcaaagcatagggacgaatatccactggtatcagcagaggacaaatggctcacctcgactgttgattaaatacgcttctgaatccatatctggaattcctagtcgcttctcagggagcggctcaggtactgacttcacactgagcattaatagcgtcgagagcgaggatatcgcagattactattgccagcaaaataacaactggccaaccaccttcggagccggcaccaaactagagctgaaaagaactgtggcagcacccagcgtctttatcttccccccaagcgacgagcagctgaaatccgggacggcgtctgttgtgtgcctgctgaacaacttttatccccgggaggccaaggtgcagtggaaagtggacaacgccctgcagtcgggaaatagccaggagtccgtcaccgaacaagatagcaaggacagcacatactccctgagcagcactctgaccctgagtaaggccgactacgaaaagcacaaggtatatgcttgtgaagtcacccaccagggcctgagtagcccagttactaagtcattcaacagaggtgagtgtgggggcggcggaagcgtggacaacaagttcaacaaggaggaatgctctgccatgcaggagatttctatgctgcccaacctgaacccgcatcagttcgctgccttcatttggtccctgatggacgacccttcccagtccgccaacctgctggccgaggccaagaagctgaacgacgcccaggctcccaag

SEQ ID NO: 99 - DNA, 1338 bp, synthetic construct; identical to SEQ ID NO: 83
  source 1..1338: mol_type = other DNA

SEQ ID NO: 100 - DNA, 1020 bp, synthetic construct
  source 1..1020: mol_type = other DNA
gatatcctgcttacacagagcccggtgattctgtcagtgagccctggcgaacgggtgagctttagttgcagggcctcgcaaagcatagggacgaatatccactggtatcagcagaggacaaatggctcacctcgactgttgattaaatacgcttctgaatccatatctggaattcctagtcgcttctcagggagcggctcaggtactgacttcacactgagcattaatagcgtcgagagcgaggatatcgcagattactattgccagcaaaataacaactggccaaccaccttcggagccggcaccaaactagagctgaaaagaactgtggcagcacccagcgtctttatcttccccccaagcgacgagcagctgaaatccgggacggcgtctgttgtgtgcctgctgaacaacttttatccccgggaggccaaggtgcagtggaaagtggacaacgccctgcagtcgggaaatagccaggagtccgtcaccgaacaagatagcaaggacagcacatactccctgagcagcactctgaccctgagtaaggccgactacgaaaagcacaaggtatatgcttgtgaagtcacccaccagggcctgagtagcccagttactaagtcattcaacagaggtgagtgtggtggaggtggaagcgtggacaacaagttcaacaaggaggaatgctctgccatgcaggagatttctatgctgcccaacctgaacccgcatcagttcgctgccttcatttggtccctgatggacgacccttcccagtccgccaacctgctggccgaggccaagaagctgaacgacgcccaggctcccaaggggggcggcggaagcgtggacaacaagttcaacaaggaggaatgctctgccatgcaggagatttctatgctgcccaacctgaacccgcatcagttcgctgccttcatttggtccctgatggacgacccttcccagtccgccaacctgctggccgaggccaagaagctgaacgacgcccaggctcccaag

SEQ ID NO: 101 - DNA, 15 bp, synthetic construct
  source 1..15: mol_type = other DNA
aggtactggctgcac

SEQ ID NO: 102 - DNA, 51 bp, synthetic construct
  source 1..51: mol_type = other DNA
gaaattaatcctagcagtggcagaaccaattataacgagaagttcaagtct

SEQ ID NO: 103 - DNA, 33 bp, synthetic construct
  source 1..33: mol_type = other DNA
tgggactatgacgaaggtacatggtttgcatat

SEQ ID NO: 104 - DNA, 33 bp, synthetic construct
  source 1..33: mol_type = other DNA
cgcgcctccgagaacatatactcctatctcgct

SEQ ID NO: 105 - DNA, 21 bp, synthetic construct
  source 1..21: mol_type = other DNA
aatgcccggaccctggttgag

SEQ ID NO: 106 - DNA, 27 bp, synthetic construct
  source 1..27: mol_type = other DNA
cagcaccattacggccccccatatacc

SEQ ID NO: 107 - DNA, 1341 bp, synthetic construct
  source 1..1341: mol_type = other DNA
caggttcagctcgtgcaatcaggcgctgaggttaaaaagccaggagccagtgtcaaagtgtcttgtaaggcctccgggtataccttcacaaggtactggctgcactgggtgagacaagcacccggtcagggccttgagtggatcggggaaattaatcctagcagtggcagaaccaattataacgagaagttcaagtctcgcgccactctgactgtagataaaagcatcagcacggcctacatggagctgtctagactgagatccgacgataccgctgtctactactgcgcgagatgggactatgacgaaggtacatggtttgcatattggggccagggaaccttggtgacagtgtcatccgctagcacaaagggtccatccgtgttccccctggctccatgttcccgctcaacctccgaatcaaccgccgcactgggctgcctggtcaaagactacttccctgagccagtgacagtgtcttggaactccggcgccctgacatctggcgtgcacacctttccagctgtgctgcagtccagcggcctgtactccctgtcttccgtggtgacagtgcctagctcttccctgggcaccaagacatatacctgcaacgtggaccataagccatccaataccaaggtggataagagggtggagagcaagtacggaccaccttgcccaccatgtccagctcctgagttcctgggcggacctagcgtgttcctgtttcctccaaagccaaaggacacactgatgatcagcagaacaccagaggtgacctgcgtggtggtggacgtgtctcaggaggatcccgaggtgcagttcaactggtacgtggatggcgtggaggtgcacaatgctaagaccaagcccagagaggagcagtttaactccacataccgcgtggtgagcgtgctgaccgtgctgcatcaggactggctgaacggcaaggagtataagtgcaaggtgtccaataagggcctgcctagctctatcgagaagacaatcagcaaggctaagggacagccaagggagccacaggtgtacaccctgcccccttctcaggaggagatgacaaagaaccaggtgtccctgacctgtctggtgaagggcttctatcccagcgacatcgctgtggagtgggagtctaatggccagcctgagaacaattacaagaccacaccacccgtgctggacagcgatggctctttctttctgtattctaggctgaccgtggataagtcccggtggcaggagggcaacgtgttctcctgcagcgtgatgcacgaagcactgcacaatcactacactcagaagagcctgtccctgtccctgggtaaa

SEQ ID NO: 108 - DNA, 642 bp, synthetic construct
  source 1..642: mol_type = other DNA
gacatccagatgacccagtcacctagcttcctgtctgcttctgtcggggacagagtgactatcacttgtcgcgcctccgagaacatatactcctatctcgcttggtaccaacagaagcccgggaaggccccaaaacttctggtatacaatgcccggaccctggttgagggcgtgccttcaaggttcagtgggagcggctccggaaccgaattcacgttgacaattagtagcctgcaaccggaggattttgcaacatactattgccagcaccattacggccccccatatacctttggacagggtacaaaggtggaaattaaacgtacggtggctgcaccatctgtcttcatcttcccgccatctgatgagcagttgaaatctggaactgcctctgttgtgtgcctgctgaataacttctatcccagagaggccaaagtacagtggaaggtggataacgccctccaatcgggtaactcccaggagagtgtcacagagcaggacagcaaggacagcacctacagcctcagcagcaccctgacgctgagcaaagcagactacgagaaacacaaagtctacgcctgcgaagtcacccatcagggcctgagttcgcccgtcacaaagagcttcaacaggggagagtgt

SEQ ID NO: 109 - DNA, 1530 bp, synthetic construct
  source 1..1530: mol_type = other DNA
caggttcagctcgtgcaatcaggcgctgaggttaaaaagccaggagccagtgtcaaagtgtcttgtaaggcctccgggtataccttcacaaggtactggctgcactgggtgagacaagcacccggtcagggccttgagtggatcggggaaattaatcctagcagtggcagaaccaattataacgagaagttcaagtctcgcgccactctgactgtagataaaagcatcagcacggcctacatggagctgtctagactgagatccgacgataccgctgtctactactgcgcgagatgggactatgacgaaggtacatggtttgcatattggggccagggaaccttggtgacagtgtcatccgctagcacaaagggtccatccgtgttccccttggctccatgttcccgctcaacctccgaatcaaccgccgcactgggctgcctggtcaaagactacttccctgagccagtgacagtgtcttggaactccggcgccctgacatctggcgtgcacacctttccagctgtgctgcagtccagcggcctgtactccctgtcttccgtggtgacagtgcctagctcttccctgggcaccaagacatatacctgcaacgtggaccataagccatccaataccaaggtggataagagggtggagagcaagtacggaccaccttgcccaccatgtccagctcctgagttcctgggcggacctagcgtgttcctgtttcctccaaagccaaaggacacactgatgatcagcagaacaccagaggtgacctgcgtggtggtggacgtgtctcaggaggatcccgaggtgcagttcaactggtatgtggacggcgtggaagtgcataatgcaaaaaccaaacccagagaagagcaattcaacagcacatacagggttgtgtcagttctcacagtgctgcaccaagactggctgaatggcaaggaatacaaatgtaaagttagcaataagggcctgccttcaagcatcgaaaagaccatcagcaaagccaaaggtcagccaagagaaccccaggtatacactttgcctccaagccaggaagagatgaccaaaaatcaggtgagcctgacctgcctggttaagggtttttacccgagcgatattgccgtggagtgggaaagcaatggccagcctgaaaacaattataagacaaccccccccgttctggactccgacggatcttttttcctatacagcagactgaccgtggataagtccaggtggcaggagggaaacgtgttcagctgttctgtgatgcatgaagccttacacaaccactatacccaaaagagcttatccctaagcctgggcaaagggggcggcggaagcgtggataacaaatttaacaaagaggtgtgcagagctatggaggaaataggaatgctgcccaacttaaacgcccaccaactggccgctttcatctggtcactgccagacgatcccagccagagcgccaatctgcttgctgaggccaaaaagctgaacgacgcccaggctcccaag

SEQ ID NO: 110 - DNA, 642 bp, synthetic construct; identical to SEQ ID NO: 108
  source 1..642: mol_type = other DNA

SEQ ID NO: 111 - DNA, 1719 bp, synthetic construct
  source 1..1719: mol_type = other DNA
caggttcagctcgtgcaatcaggcgctgaggttaaaaagccaggagccagtgtcaaagtgtcttgtaaggcctccgggtataccttcacaaggtactggctgcactgggtgagacaagcacccggtcagggccttgagtggatcggggaaattaatcctagcagtggcagaaccaattataacgagaagttcaagtctcgcgccactctgactgtagataaaagcatcagcacggcctacatggagctgtctagactgagatccgacgataccgctgtctactactgcgcgagatgggactatgacgaaggtacatggtttgcatattggggccagggaaccttggtgacagtgtcatccgctagcacaaagggtccatccgtgttccccctggctccatgttcccgctcaacctccgaatcaaccgccgcactgggctgcctggtcaaagactacttccctgagccagtgacagtgtcttggaactccggcgccctgacatctggcgtgcacacctttccagctgtgctgcagtccagcggcctgtactccctgtcttccgtggtgacagtgcctagctcttccctgggcaccaagacatatacctgcaacgtggaccataagccatccaataccaaggtggataagagggtggagagcaagtacggaccaccttgcccaccatgtccagctcctgagttcctgggcggacctagcgtgttcctgtttcctccaaagccaaaggacacactgatgatcagcagaacaccagaggtgacctgcgtggtggtggacgtgtctcaggaggatcccgaggtgcagttcaactggtacgtggatggcgtggaggtgcacaatgctaagaccaagcccagagaggagcagtttaactccacataccgcgtggtgagcgtgctgaccgtgctgcatcaggactggctgaacggcaaggagtataagtgcaaggtgtccaataagggcctgcctagctctatcgagaagacaatcagcaaggctaagggacagccaagggagccacaggtgtacaccctgcccccttctcaggaggagatgacaaagaaccaggtgtccctgacctgtctggtgaagggcttctatcccagcgacatcgctgtggagtgggagtctaatggccagcctgagaacaattacaagaccacaccacccgtgctggacagcgatggctctttctttctgtattctaggctgaccgtggataagtcccggtggcaggagggcaacgtgttctcctgcagcgtgatgcacgaagcactgcacaatcactacactcagaagagcctgtccctgtccctgggtaaaggtggaggtggaagcgtggataacaaatttaacaaagaggtgtgcagagctatggaggaaataggaatgctgcccaacttaaacgcccaccaactggccgctttcatctggtcactgccagacgatcccagccagagcgccaatctgcttgctgaggccaaaaagctgaatgacgcccaggcccctaaggggggcggcggaagcgtggataacaaatttaacaaagaggtgtgcagagctatggaggaaataggaatgctgcccaacttaaacgcccaccaactggccgctttcatctggtcactgccagacgatcccagccagagcgccaatctgcttgctgaggccaaaaagctgaacgacgcccaggcccctaag

SEQ ID NO: 112 - DNA, 642 bp, synthetic construct; identical to SEQ ID NO: 108
  source 1..642: mol_type = other DNA

SEQ ID NO: 113 - DNA, 1530 bp, synthetic construct; identical to SEQ ID NO: 109
  source 1..1530: mol_type = other DNA

SEQ ID NO: 114 - DNA, 831 bp, synthetic construct
  source 1..831: mol_type = other DNA
gacatccagatgacccagtcacctagcttcctgtctgcttctgtcggggacagagtgactatcacttgtcgcgcctccgagaacatatactcctatctcgcttggtaccaacagaagcccgggaaggccccaaaacttctggtatacaatgcccggaccctggttgagggcgtgccttcaaggttcagtgggagcggctccggaaccgaattcacgttgacaattagtagcctgcaaccggaggattttgcaacatactattgccagcaccattacggccccccatatacctttggacagggtacaaaggtggaaattaaacgtacggtggctgcaccatctgtcttcatcttcccgccatctgatgagcagttgaaatctggaactgcctctgttgtgtgcctgctgaataacttctatcccagagaggccaaagtacagtggaaggtggataacgccctccaatcgggtaactcccaggagagtgtcacagagcaggacagcaaggacagcacctacagcctcagcagcaccctgacgctgagcaaagcagactacgagaaacacaaagtctacgcctgcgaagtcacccatcagggcctgagttcgcccgtcacaaagagcttcaacaggggagagtgtggcggaggcggctctgtggacaacaagttcaacaaggaggtttgccgtgccatggaagagattggtatgctgcccaacctgaacgctcatcagctggctgccttcatttggtccctgccggacgacccttcccagtccgccaacctgctggccgaggccaagaagctgaacgacgcccaggctcccaag

SEQ ID NO: 115 - DNA, 1341 bp, synthetic construct; identical to SEQ ID NO: 107
  source 1..1341: mol_type = other DNA

SEQ ID NO: 116 - DNA, 1020 bp, synthetic construct
  source 1..1020: mol_type = other DNA
gacatccagatgacccagtcacctagcttcctgtctgcttctgtcggggacagagtgactatcacttgtcgcgcctccgagaacatatactcctatctcgcttggtaccaacagaagcccgggaaggccccaaaacttctggtatacaatgcccggaccctggttgagggcgtgccttcaaggttcagtgggagcggctccggaaccgaattcacgttgacaattagtagcctgcaaccggaggattttgcaacatactattgccagcaccattacggccccccatatacctttggacagggtacaaaggtggaaattaaacgtacggtggctgcaccatctgtcttcatcttcccgccatctgatgagcagttgaaatctggaactgcctctgttgtgtgcctgctgaataacttctatcccagagaggccaaagtacagtggaaggtggataacgccctccaatcgggtaactcccaggagagtgtcacagagcaggacagcaaggacagcacctacagcctcagcagcaccctgacgctgagcaaagcagactacgagaaacacaaagtctacgcctgcgaagtcacccatcagggcctgagttcgcccgtcacaaagagcttcaacaggggagagtgtggtggaggtggaagcgtggataacaaatttaacaaagaggtgtgcagagctatggaggaaataggaatgctgcccaacttaaacgcccaccaactggccgctttcatctggtcactgccagacgatcccagccagagcgccaatctgcttgctgaggccaaaaagctgaatgacgcccaggcccctaaggggggcggcggaagcgtggataacaaatttaacaaagaggtgtgcagagctatggaggaaataggaatgctgcccaacttaaacgcccaccaactggccgctttcatctggtcactgccagacgatcccagccagagcgccaatctgcttgctgaggccaaaaagctgaacgacgcccaggcccctaag

SEQ ID NO: 117 - DNA, 1530 bp, synthetic construct
  source 1..1530: mol_type = other DNA
caggttcagctcgtgcaatcaggcgctgaggttaaaaagccaggagccagtgtcaaagtgtcttgtaaggcctccgggtataccttcacaaggtactggctgcactgggtgagacaagcacccggtcagggccttgagtggatcggggaaattaatcctagcagtggcagaaccaattataacgagaagttcaagtctcgcgccactctgactgtagataaaagcatcagcacggcctacatggagctgtctagactgagatccgacgataccgctgtctactactgcgcgagatgggactatgacgaaggtacatggtttgcatattggggccagggaaccttggtgacagtgtcatccgcatcaaccaagggacccagcgtgtttcccctggctccctgcagcagaagtaccagcgagagcaccgcggccctgggctgccttgtgaaagactactttcctgagccggtgaccgtgtcatggaattcgggcgccctgactagcggagtacacaccttcccggccgtactgcagagcagcggcctgtacagcctgagctccgtggtgacggtgcccagctctagcctaggtacgaagacctacacttgtaacgtggatcataagcccagcaacaccaaggttgacaagcgggtggaaagcaagtatggtccgccatgtccaccatgccccgcacctgagtttctggggggcccaagcgtattcctttttcccccaaaacctaaagataccctgatgatttcccgtactcccgaggtgacgtgtgtggtggtggatgtgagccaggaggatccagaggtccagttcaactggtatgtggacggcgtggaagtgcataatgcaaaaaccaaacccagagaagagcaattcaacagcacatacagggttgtgtcagttctcacagtgctgcaccaagactggctgaatggcaaggaatacaaatgtaaagttagcaataagggcctgccttcaagcatcgaaaagaccatcagcaaagccaaaggtcagccaagagaaccccaggtatacactttgcctccaagccaggaagagatgaccaaaaatcaggtgagcctgacctgcctggttaagggtttttacccgagcgatattgccgtggagtgggaaagcaatggccagcctgaaaacaattataagacaaccccccccgttctggactccgacggatcttttttcctatacagcagactgaccgtggataagtccaggtggcaggagggaaacgtgttcagctgttctgtgatgcatgaagccttacacaaccactatacccaaaagagcttatccctaagcctgggcaaagggggcggcggaagcgtggacaacaagttcaacaaggaggaatgctctgccatgcaggagatttctatgctgcccaacctgaacccgcatcagttcgctgccttcatttggtccctgatggacgacccttcccagtccgccaacctgctggccgaggccaagaagctgaacgacgcccaggctcccaag

SEQ ID NO: 118 - DNA, 642 bp, synthetic construct; identical to SEQ ID NO: 108
  source 1..642: mol_type = other DNA

SEQ ID NO: 119 - DNA, 1719 bp, synthetic construct
  source 1..1719: mol_type = other DNA
caggttcagctcgtgcaatcaggcgctgaggttaaaaagccaggagccagtgtcaaagtgtcttgtaaggcctccgggtataccttcacaaggtactggctgcactgggtgagacaagcacccggtcagggccttgagtggatcggggaaattaatcctagcagtggcagaaccaattataacgagaagttcaagtctcgcgccactctgactgtagataaaagcatcagcacggcctacatggagctgtctagactgagatccgacgataccgctgtctactactgcgcgagatgggactatgacgaaggtacatggtttgcatattggggccagggaaccttggtgacagtgtcatccgctagcacaaagggtccatccgtgttccccctggctccatgttcccgctcaacctccgaatcaaccgccgcactgggctgcctggtcaaagactacttccctgagccagtgacagtgtcttggaactccggcgccctgacatctggcgtgcacacctttccagctgtgctgcagtccagcggcctgtactccctgtcttccgtggtgacagtgcctagctcttccctgggcaccaagacatatacctgcaacgtggaccataagccatccaataccaaggtggataagagggtggagagcaagtacggaccaccttgcccaccatgtccagctcctgagttcctgggcggacctagcgtgttcctgtttcctccaaagccaaaggacacactgatgatcagcagaacaccagaggtgacctgcgtggtggtggacgtgtctcaggaggatcccgaggtgcagttcaactggtacgtggatggcgtggaggtgcacaatgctaagaccaagcccagagaggagcagtttaactccacataccgcgtggtgagcgtgctgaccgtgctgcatcaggactggctgaacggcaaggagtataagtgcaaggtgtccaataagggcctgcctagctctatcgagaagacaatcagcaaggctaagggacagccaagggagccacaggtgtacaccctgcccccttctcaggaggagatgacaaagaaccaggtgtccctgacctgtctggtgaagggcttctatcccagcgacatcgctgtggagtgggagtctaatggccagcctgagaacaattacaagaccacaccacccgtgctggacagcgatggctctttctttctgtattctaggctgaccgtggataagtcccggtggcaggagggcaacgtgttctcctgcagcgtgatgcacgaagcactgcacaatcactacactcagaagagcctgtccctgtccctgggtaaaggtggaggtggaagcgtggacaacaagttcaacaaggaggaatgctctgccatgcaggagatttctatgctgcccaacctgaacccgcatcagttcgctgccttcatttggtccctgatggacgacccttcccagtccgccaacctgctggccgaggccaagaagctgaacgacgcccaggctcccaaggggggcggcggaagcgtggacaacaagttcaacaaggaggaatgctctgccatgcaggagatttctatgctgcccaacctgaacccgcatcagttcgctgccttcatttggtccctgatggacgacccttcccagtccgccaacctgctggccgaggccaagaagctgaacgacgcccaggctcccaag

SEQ ID NO: 120 - DNA, 642 bp, synthetic construct; identical to SEQ ID NO: 108
  source 1..642: mol_type = other DNA

SEQ ID NO: 121 - DNA, 1530 bp, synthetic construct; identical to SEQ ID NO: 117
  source 1..1530: mol_type = other DNA

SEQ ID NO: 122 - DNA, 831 bp, synthetic construct
  source 1..831: mol_type = other DNA
gacatccagatgacccagtcacctagcttcctgtctgcttctgtcggggacagagtgactatcacttgtcgcgcctccgagaacatatactcctatctcgcttggtaccaacagaagcccgggaaggccccaaaacttctggtatacaatgcccggaccctggttgagggcgtgccttcaaggttcagtgggagcggctccggaaccgaattcacgttgacaattagtagcctgcaaccggaggattttgcaacatactattgccagcaccattacggccccccatatacctttggacagggtacaaaggtggaaattaaacgtacggtggctgcaccatctgtcttcatcttcccgccatctgatgagcagttgaaatctggaactgcctctgttgtgtgcctgctgaataacttctatcccagagaggccaaagtacagtggaaggtggataacgccctccaatcgggtaactcccaggagagtgtcacagagcaggacagcaaggacagcacctacagcctcagcagcaccctgacgctgagcaaagcagactacgagaaacacaaagtctacgcctgcgaagtcacccatcagggcctgagttcgcccgtcacaaagagcttcaacaggggagagtgtggcggaggcggctctgtggacaacaagttcaacaaggaggaatgctctgccatgcaggagatttctatgctgcccaacctgaacccgcatcagttcgctgccttcatttggtccctgatggacgacccttcccagtccgccaacctgctggccgaggccaagaagctgaacgacgcccaggctcccaag

SEQ ID NO: 123 - DNA, 1341 bp, synthetic construct; identical to SEQ ID NO: 107
  source 1..1341: mol_type = other DNA

SEQ ID NO: 124 - DNA, 1020 bp, synthetic construct
  source 1..1020: mol_type = other DNA
gacatccagatgacccagtcacctagcttcctgtctgcttctgtcggggacagagtgactatcacttgtcgcgcctccgagaacatatactcctatctcgcttggtaccaacagaagcccgggaaggccccaaaacttctggtatacaatgcccggaccctggttgagggcgtgccttcaaggttcagtgggagcggctccggaaccgaattcacgttgacaattagtagcctgcaaccggaggattttgcaacatactattgccagcaccattacggccccccatatacctttggacagggtacaaaggtggaaattaaacgtacggtggctgcaccatctgtcttcatcttcccgccatctgatgagcagttgaaatctggaactgcctctgttgtgtgcctgctgaataacttctatcccagagaggccaaagtacagtggaaggtggataacgccctccaatcgggtaactcccaggagagtgtcacagagcaggacagcaaggacagcacctacagcctcagcagcaccctgacgctgagcaaagcagactacgagaaacacaaagtctacgcctgcgaagtcacccatcagggcctgagttcgcccgtcacaaagagcttcaacaggggagagtgtggtggaggtggaagcgtggacaacaagttcaacaaggaggaatgctctgccatgcaggagatttctatgctgcccaacctgaacccgcatcagttcgctgccttcatttggtccctgatggacgacccttcccagtccgccaacctgctggccgaggccaagaagctgaacgacgcccaggctcccaaggggggcggcggaagcgtggacaacaagttcaacaaggaggaatgctctgccatgcaggagatttctatgctgcccaacctgaacccgcatcagttcgctgccttcatttggtccctgatggacgacccttcccagtccgccaacctgctggccgaggccaagaagctgaacgacgcccaggctcccaag

SEQ ID NO: 125 - DNA, 15 bp, synthetic construct
  source 1..15: mol_type = other DNA
gaatacaccatccac

SEQ ID NO: 126 - DNA, 51 bp, synthetic construct
  source 1..51: mol_type = other DNA
aacattaatcccaacaatgggggcacaacttacaatcaaaagttcgaggac

SEQ ID NO: 127 - DNA, 18 bp, synthetic construct
  source 1..18: mol_type = other DNA
gggtggaactttgattat

SEQ ID NO: 128 - DNA, 33 bp, synthetic construct
  source 1..33: mol_type = other DNA
aaggcctctcaggacgtcggaacagccgttgac

SEQ ID NO: 129 - DNA, 21 bp, synthetic construct
  source 1..21: mol_type = other DNA
tgggcaagcaccagacacacc

SEQ ID NO: 130 - DNA, 27 bp, synthetic construct
  source 1..27: mol_type = other DNA
cagcagtacaacagttaccctctgaca

SEQ ID NO: 131 - DNA, 1326 bp, synthetic construct
  source 1..1326: mol_type = other DNA
gaagtgcagctggttcagagcggtcccgaggtaaagaaaccaggagcaactgtgaagattagctgtaagacatctggatataccttcacagaatacaccatccactgggtgaaacaggcccctggcaaaggcctggagtggatcggcaacattaatcccaacaatgggggcacaacttacaatcaaaagttcgaggacaaagccacacttacagtcgacaagtccaccgacaccgcttacatggagttgagttcccttcggtcagaggatactgccgtgtattactgcgctgccgggtggaactttgattattggggccagggtaccctgctcacggtctctagcgcatcaaccaagggacccagcgtgtttcccctggctccctgcagcagaagtaccagcgagagcaccgcggccctgggctgccttgtgaaagactactttcctgagccggtgaccgtgtcatggaattcgggcgccctgactagcggagtacacaccttcccggccgtactgcagagcagcggcctgtacagcctgagctccgtggtgacggtgcccagctctagcctaggtacgaagacctacacttgtaacgtggatcataagcccagcaacaccaaggttgacaagcgggtggaaagcaagtatggcccgccatgtccaccatgccccgcacctgagtttctggggggcccaagcgtattcctttttcccccaaaacctaaagataccctgatgatttcccgtactcccgaggtgacgtgtgtggtggtggatgtgagccaggaggatccagaggtccagttcaactggtatgtggacggcgtggaagtgcataatgcaaaaaccaaacccagagaagagcaattcaacagcacatacagggttgtgtcagttctcacagtgctgcaccaagactggctgaatggcaaggaatacaaatgtaaagttagcaataagggcctgccttcaagcatcgaaaagaccatcagcaaagccaaaggtcagccaagagaaccccaggtatacactttgcctccaagccaggaagagatgaccaaaaatcaggtgagcctgacctgcctggttaagggtttttacccgagcgatattgccgtggagtgggaaagcaatggccagcctgaaaacaattataagacaaccccccccgttctggactccgacggatcttttttcctatacagcagactgaccgtggataagtccaggtggcaggagggaaacgtgttcagctgttctgtgatgcatgaagccttacacaaccactatacccaaaagagcttatccctaagcctgggcaaa

SEQ ID NO: 132 - DNA, 642 bp, synthetic construct
  source 1..642: mol_type = other DNA
gatatccagatgacacaaagcccgagttcactgtcgacctccgtgggtgacagagtgactctcacgtgcaaggcctctcaggacgtcggaacagccgttgactggtaccagcagaagcctggcccctctccaaaacttctgatttattgggcaagcaccagacacaccggcataccctcaagattctccgggagcggatccggcactgactttacgttaacaatctcttccttgcaaccagaagatttcgctgattattattgtcagcagtacaacagttaccctctgacatttggacccgggaccaaagtcgatattaagagaactgtggcagcacccagcgtctttatcttccccccaagcgacgagcagctgaaatccgggacggcgtctgttgtgtgcctgctgaacaacttttatccccgggaggccaaggtgcagtggaaagtggacaacgccctgcagtcgggaaatagccaggagtccgtcaccgaacaagatagcaaggacagcacatactccctgagcagcactctgaccctgagtaaggccgactacgaaaagcacaaggtatatgcttgtgaagtcacccaccagggcctgagtagcccagttactaagtcattcaacagaggtgagtgt

SEQ ID NO: 133 - DNA, 1515 bp, synthetic construct
  source 1..1515: mol_type = other DNA
gaagtgcagctggttcagagcggtcccgaggtaaagaaaccaggagcaactgtgaagattagctgtaagacatctggatataccttcacagaatacaccatccactgggtgaaacaggcccctggcaaaggcctggagtggatcggcaacattaatcccaacaatgggggcacaacttacaatcaaaagttcgaggacaaagccacacttacagtcgacaagtccaccgacaccgcttacatggagttgagttcccttcggtcagaggatactgccgtgtattactgcgctgccgggtggaactttgattattggggccagggtaccctgctcacggtctctagcgcatcaaccaagggacccagcgtgtttcccctggctccctgcagcagaagtaccagcgagagcaccgcggccctgggctgccttgtgaaagactactttcctgagccggtgaccgtgtcatggaattcgggcgccctgactagcggagtacacaccttcccggccgtactgcagagcagcggcctgtacagcctgagctccgtggtgacggtgcccagctctagcctaggtacgaagacctacacttgtaacgtggatcataagcccagcaacaccaaggttgacaagcgggtggaaagcaagtatggcccgccatgtccaccatgccccgcacctgagtttctggggggcccaagcgtattcctttttcccccaaaacctaaagataccctgatgatttcccgtactcccgaggtgacgtgtgtggtggtggatgtgagccaggaggatccagaggtccagttcaactggtatgtggacggcgtggaagtgcataatgcaaaaaccaaacccagagaagagcaattcaacagcacatacagggttgtgtcagttctcacagtgctgcaccaagactggctgaatggcaaggaatacaaatgtaaagttagcaataagggcctgccttcaagcatcgaaaagaccatcagcaaagccaaaggtcagccaagagaaccccaggtatacactttgcctccaagccaggaagagatgaccaaaaatcaggtgagcctgacctgcctggttaagggtttttacccgagcgatattgccgtggagtgggaaagcaatggccagcctgaaaacaattataagacaaccccccccgttctggactccgacggatcttttttcctatacagcagactgaccgtggataagtccaggtggcaggagggaaacgtgttcagctgttctgtgatgcatgaagccttacacaaccactatacccaaaagagcttatccctaagcctgggcaaagggggcggcggaagcgtggataacaaatttaacaaagaggtgtgcagagctatggaggaaataggaatgctgcccaacttaaacgcccaccaactggccgctttcatctggtcactgccagacgatcccagccagagcgccaatctgcttgctgaggccaaaaagctgaacgacgcccaggcccctaag

SEQ ID NO: 134 - DNA, 642 bp, synthetic construct; identical to SEQ ID NO: 132
  source 1..642: mol_type = other DNA

SEQ ID NO: 135 - DNA, 1704 bp, synthetic construct
  source 1..1704: mol_type = other DNA
gaagtgcagctggttcagagcggtcccgaggtaaagaaaccaggagcaactgtgaagattagctgtaagacatctggatataccttcacagaatacaccatccactgggtgaaacaggcccctggcaaaggcctggagtggatcggcaacattaatcccaacaatgggggcacaacttacaatcaaaagttcgaggacaaagccacacttacagtcgacaagtccaccgacaccgcttacatggagttgagttcccttcggtcagaggatactgccgtgtattactgcgctgccgggtggaactttgattattggggccagggtaccctgctcacggtctctagcgcatcaaccaagggacccagcgtgtttcccctggctccctgcagcagaagtaccagcgagagcaccgcggccctgggctgccttgtgaaagactactttcctgagccggtgaccgtgtcatggaattcgggcgccctgactagcggagtacacaccttcccggccgtactgcagagcagcggcctgtacagcctgagctccgtggtgacggtgcccagctctagcctaggtacgaagacctacacttgtaacgtggatcataagcccagcaacaccaaggttgacaagcgggtggaaagcaagtatggcccgccatgtccaccatgccccgcacctgagtttctggggggcccaagcgtattcctttttcccccaaaacctaaagataccctgatgatttcccgtactcccgaggtgacgtgtgtggtggtggatgtgagccaggaggatccagaggtccagttcaactggtatgtggacggcgtggaagtgcataatgcaaaaaccaaacccagagaagagcaattcaacagcacatacagggttgtgtcagttctcacagtgctgcaccaagactggctgaatggcaaggaatacaaatgtaaagttagcaataagggcctgccttcaagcatcgaaaagaccatcagcaaagccaaaggtcagccaagagaaccccaggtatacactttgcctccaagccaggaagagatgaccaaaaatcaggtgagcctgacctgcctggttaagggtttttacccgagcgatattgccgtggagtgggaaagcaatggccagcctgaaaacaattataagacaaccccccccgttctggactccgacggatcttttttcctatacagcagactgaccgtggataagtccaggtggcaggagggaaacgtgttcagctgttctgtgatgcatgaagccttacacaaccactatacccaaaagagcttatccctaagcctgggcaaaggtggaggtggaagcgtggataacaaatttaacaaagaggtgtgcagagctatggaggaaataggaatgctgcccaacttaaacgcccaccaactggccgctttcatctggtcactgccagacgatcccagccagagcgccaatctgcttgctgaggccaaaaagctgaatgacgcccaggcccctaaggggggcggcggaagcgtggataacaaatttaacaaagaggtgtgcagagctatggaggaaataggaatgctgcccaacttaaacgcccaccaactggccgctttcatctggtcactgccagacgatcccagccagagcgccaatctgcttgctgaggccaaaaagctgaacgacgcccaggcccctaag

SEQ ID NO: 136 - DNA, 642 bp, synthetic construct; identical to SEQ ID NO: 132
  source 1..642: mol_type = other DNA

SEQ ID NO: 137 - DNA, 1515 bp, synthetic construct; identical to SEQ ID NO: 133
  source 1..1515: mol_type = other DNA

SEQ ID NO: 138 - DNA, 831 bp, synthetic construct
  source 1..831: mol_type = other DNA
gatatccagatgacacaaagcccgagttcactgtcgacctccgtgggtgacagagtgactctcacgtgcaaggcctctcaggacgtcggaacagccgttgactggtaccagcagaagcctggcccctctccaaaacttctgatttattgggcaagcaccagacacaccggcataccctcaagattctccgggagcggatccggcactgactttacgttaacaatctcttccttgcaaccagaagatttcgctgattattattgtcagcagtacaacagttaccctctgacatttggacccgggaccaaagtcgatattaagagaactgtggcagcacccagcgtctttatcttccccccaagcgacgagcagctgaaatccgggacggcgtctgttgtgtgcctgctgaacaacttttatccccgggaggccaaggtgcagtggaaagtggacaacgccctgcagtcgggaaatagccaggagtccgtcaccgaacaagatagcaaggacagcacatactccctgagcagcactctgaccctgagtaaggccgactacgaaaagcacaaggtatatgcttgtgaagtcacccaccagggcctgagtagcccagttactaagtcattcaacagaggtgagtgtgggggcggcggaagcgtggataacaaatttaacaaagaggtgtgcagagctatggaggaaataggaatgctgcccaacttaaacgcccaccaactggccgctttcatctggtcactgccagacgatcccagccagagcgccaatctgcttgctgaggccaaaaagctgaacgacgcccaggcccctaag

SEQ ID NO: 139 - DNA, 1326 bp, synthetic construct; identical to SEQ ID NO: 131
  source 1..1326: mol_type = other DNA

SEQ ID NO: 140 - DNA, 1020 bp, synthetic construct
  source 1..1020: mol_type = other DNA
gatatccagatgacacaaagcccgagttcactgtcgacctccgtgggtgacagagtgactctcacgtgcaaggcctctcaggacgtcggaacagccgttgactggtaccagcagaagcctggcccctctccaaaacttctgatttattgggcaagcaccagacacaccggcataccctcaagattctccgggagcggatccggcactgactttacgttaacaatctcttccttgcaaccagaagatttcgctgattattattgtcagcagtacaacagttaccctctgacatttggacccgggaccaaagtcgatattaagagaactgtggcagcacccagcgtctttatcttccccccaagcgacgagcagctgaaatccgggacggcgtctgttgtgtgcctgctgaacaacttttatccccgggaggccaaggtgcagtggaaagtggacaacgccctgcagtcgggaaatagccaggagtccgtcaccgaacaagatagcaaggacagcacatactccctgagcagcactctgaccctgagtaaggccgactacgaaaagcacaaggtatatgcttgtgaagtcacccaccagggcctgagtagcccagttactaagtcattcaacagaggtgagtgtggtggaggtggaagcgtggataacaaatttaacaaagaggtgtgcagagctatggaggaaataggaatgctgcccaacttaaacgcccaccaactggccgctttcatctggtcactgccagacgatcccagccagagcgccaatctgcttgctgaggccaaaaagctgaatgacgcccaggcccctaaggggggcggcggaagcgtggataacaaatttaacaaagaggtgtgcagagctatggaggaaataggaatgctgcccaacttaaacgcccaccaactggccgctttcatctggtcactgccagacgatcccagccagagcgccaatctgcttgctgaggccaaaaagctgaacgacgcccaggcccctaag

SEQ ID NO: 141 - DNA, 1515 bp, synthetic construct
  source 1..1515: mol_type = other DNA
gaagtgcagctggttcagagcggtcccgaggtaaagaaaccaggagcaactgtgaagattagctgtaagacatctggatataccttcacagaatacaccatccactgggtgaaacaggcccctggcaaaggcctggagtggatcggcaacattaatcccaacaatgggggcacaacttacaatcaaaagttcgaggacaaagccacacttacagtcgacaagtccaccgacaccgcttacatggagttgagttcccttcggtcagaggatactgccgtgtattactgcgctgccgggtggaactttgattattggggccagggtaccctgctcacggtctctagcgcatcaaccaagggacccagcgtgtttcccctggctccctgcagcagaagtaccagcgagagcaccgcggccctgggctgccttgtgaaagactactttcctgagccggtgaccgtgtcatggaattcgggcgccctgactagcggagtacacaccttcccggccgtactgcagagcagcggcctgtacagcctgagctccgtggtgacggtgcccagctctagcctaggtacgaagacctacacttgtaacgtggatcataagcccagcaacaccaaggttgacaagcgggtggaaagcaagtatggcccgccatgtccaccatgccccgcacctgagtttctggggggcccaagcgtattcctttttcccccaaaacctaaagataccctgatgatttcccgtactcccgaggtgacgtgtgtggtggtggatgtgagccaggaggatccagaggtccagttcaactggtatgtggacggcgtggaagtgcataatgcaaaaaccaaacccagagaagagcaattcaacagcacatacagggttgtgtcagttctcacagtgctgcaccaagactggctgaatggcaaggaatacaaatgtaaagttagcaataagggcctgccttcaagcatcgaaaagaccatcagcaaagccaaaggtcagccaagagaaccccaggtatacactttgcctccaagccaggaagagatgaccaaaaatcaggtgagcctgacctgcctggttaagggtttttacccgagcgatattgccgtggagtgggaaagcaatggccagcctgaaaacaattataagacaaccccccccgttctggactccgacggatcttttttcctatacagcagactgaccgtggataagtccaggtggcaggagggaaacgtgttcagctgttctgtgatgcatgaagccttacacaaccactatacccaaaagagcttatccctaagcctgggcaaagggggcggcggaagcgtggacaacaagttcaacaaggaggaatgctctgccatgcaggagatttctatgctgcccaacctgaacccgcatcagttcgctgccttcatttggtccctgatggacgacccttcccagtccgccaacctgctggccgaggccaagaagctgaacgacgcccaggctcccaag

SEQ ID NO: 142 - DNA, 642 bp, synthetic construct; identical to SEQ ID NO: 132
  source 1..642: mol_type = other DNA

SEQ ID NO: 143 - DNA, 1704 bp, synthetic construct
  source 1..1704: mol_type = other DNA
gaagtgcagctggttcagagcggtcccgaggtaaagaaaccaggagcaactgtgaagattagctgtaagacatctggatataccttcacagaatacaccatccactgggtgaaacaggcccctggcaaaggcctggagtggatcggcaacattaatcccaacaatgggggcacaacttacaatcaaaagttcgaggacaaagccacacttacagtcgacaagtccaccgacaccgcttacatggagttgagttcccttcggtcagaggatactgccgtgtattactgcgctgccgggtggaactttgattattggggccagggtaccctgctcacggtctctagcgcatcaaccaagggacccagcgtgtttcccctggctccctgcagcagaagtaccagcgagagcaccgcggccctgggctgccttgtgaaagactactttcctgagccggtgaccgtgtcatggaattcgggcgccctgactagcggagtacacaccttcccggccgtactgcagagcagcggcctgtacagcctgagctccgtggtgacggtgcccagctctagcctaggtacgaagacctacacttgtaacgtggatcataagcccagcaacaccaaggttgacaagcgggtggaaagcaagtatggcccgccatgtccaccatgccccgcacctgagtttctggggggcccaagcgtattcctttttcccccaaaacctaaagataccctgatgatttcccgtactcccgaggtgacgtgtgtggtggtggatgtgagccaggaggatccagaggtccagttcaactggtatgtggacggcgtggaagtgcataatgcaaaaaccaaacccagagaagagcaattcaacagcacatacagggttgtgtcagttctcacagtgctgcaccaagactggctgaatggcaaggaatacaaatgtaaagttagcaataagggcctgccttcaagcatcgaaaagaccatcagcaaagccaaaggtcagccaagagaaccccaggtatacactttgcctccaagccaggaagagatgaccaaaaatcaggtgagcctgacctgcctggttaagggtttttacccgagcgatattgccgtggagtgggaaagcaatggccagcctgaaaacaattataagacaaccccccccgttctggactccgacggatcttttttcctatacagcagactgaccgtggataagtccaggtggcaggagggaaacgtgttcagctgttctgtgatgcatgaagccttacacaaccactatacccaaaagagcttatccctaagcctgggcaaaggtggaggtggaagcgtggacaacaagttcaacaaggaggaatgctctgccatgcaggagatttctatgctgcccaacctgaacccgcatcagttcgctgccttcatttggtccctgatggacgacccttcccagtccgccaacctgctggccgaggccaagaagctgaacgacgcccaggctcccaaggggggcggcggaagcgtggacaacaagttcaacaaggaggaatgctctgccatgcaggagatttctatgctgcccaacctgaacccgcatcagttcgctgccttcatttggtccctgatggacgacccttcccagtccgccaacctgctggccgaggccaagaagctgaacgacgcccaggctcccaag

SEQ ID NO: 144 - DNA, 642 bp, synthetic construct; identical to SEQ ID NO: 132
  source 1..642: mol_type = other DNA

SEQ ID NO: 145 - DNA, 1515 bp, synthetic construct; identical to SEQ ID NO: 141
  source 1..1515: mol_type = other DNA

SEQ ID NO: 146 - DNA, 831 bp, synthetic construct
  source 1..831: mol_type = other DNA
gatatccagatgacacaaagcccgagttcactgtcgacctccgtgggtgacagagtgactctcacgtgcaaggcctctcaggacgtcggaacagccgttgactggtaccagcagaagcctggcccctctccaaaacttctgatttattgggcaagcaccagacacaccggcataccctcaagattctccgggagcggatccggcactgactttacgttaacaatctcttccttgcaaccagaagatttcgctgattattattgtcagcagtacaacagttaccctctgacatttggacccgggaccaaagtcgatattaagagaactgtggcagcacccagcgtctttatcttccccccaagcgacgagcagctgaaatccgggacggcgtctgttgtgtgcctgctgaacaacttttatccccgggaggccaaggtgcagtggaaagtggacaacgccctgcagtcgggaaatagccaggagtccgtcaccgaacaagatagcaaggacagcacatactccctgagcagcactctgaccctgagtaaggccgactacgaaaagcacaaggtatatgcttgtgaagtcacccaccagggcctgagtagcccagttactaagtcattcaacagaggtgagtgtgggggcggcggaagcgtggacaacaagttcaacaaggaggaatgctctgccatgcaggagatttctatgctgcccaacctgaacccgcatcagttcgctgccttcatttggtccctgatggacgacccttcccagtccgccaacctgctggccgaggccaagaagctgaacgacgcccaggctcccaag

SEQ ID NO: 147 - DNA, 1326 bp, synthetic construct; identical to SEQ ID NO: 131
  source 1..1326: mol_type = other DNA

SEQ ID NO: 148 - DNA, 1020 bp, synthetic construct
  source 1..1020: mol_type = other DNA
gatatccagatgacacaaagcccgagttcactgtcgacctccgtgggtgacagagtgactctcacgtgcaaggcctctcaggacgtcggaacagccgttgactggtaccagcagaagcctggcccctctccaaaacttctgatttattgggcaagcaccagacacaccggcataccctcaagattctccgggagcggatccggcactgactttacgttaacaatctcttccttgcaaccagaagatttcgctgattattattgtcagcagtacaacagttaccctctgacatttggacccgggaccaaagtcgatattaagagaactgtggcagcacccagcgtctttatcttccccccaagcgacgagcagctgaaatccgggacggcgtctgttgtgtgcctgctgaacaacttttatccccgggaggccaaggtgcagtggaaagtggacaacgccctgcagtcgggaaatagccaggagtccgtcaccgaacaagatagcaaggacagcacatactccctgagcagcactctgaccctgagtaaggccgactacgaaaagcacaaggtatatgcttgtgaagtcacccaccagggcctgagtagcccagttactaagtcattcaacagaggtgagtgtggtggaggtggaagcgtggacaacaagttcaacaaggaggaatgctctgccatgcaggagatttctatgctgcccaacctgaacccgcatcagttcgctgccttcatttggtccctgatggacgacccttcccagtccgccaacctgctggccgaggccaagaagctgaacgacgcccaggctcccaaggggggcggcggaagcgtggacaacaagttcaacaaggaggaatgctctgccatgcaggagatttctatgctgcccaacctgaacccgcatcagttcgctgccttcatttggtccctgatggacgacccttcccagtccgccaacctgctggccgaggccaagaagctgaacgacgcccaggctcccaag